European Patent Application EP 4 339 210 A1, published March 20, 2024. Title: COMBINATION TREATMENT WITH ANTI CD300C ANTIBODY. Applicant: CentricsBio, Inc. The sequence listing filed with the application follows.

SEQUENCE LISTING (408 sequences)

SEQ ID NO: 1 - DNA, 30 bp, Artificial Sequence
  CK1 Heavy Chain CDR1
ttcagccgctatgccatgacctgggttcgc

SEQ ID NO: 2 - DNA, 45 bp, Artificial Sequence
  CK1 Heavy Chain CDR2
agcagcatgagcggcaccggcggcaccacctattatgccgatagc

SEQ ID NO: 3 - DNA, 36 bp, Artificial Sequence
  CK1 Heavy Chain CDR3
tactgtgcccgcggcgcctatggctttgatcattgg

SEQ ID NO: 4 - DNA, 41 bp, Artificial Sequence
  CK1 Light Chain CDR1
tgccgcgccagccagagcatcggcaactatctgaactggta

SEQ ID NO: 5 - DNA, 36 bp, Artificial Sequence
  CK1 Light Chain CDR2
ctgatctatgatgccagcaacctggaaaccggcatc

SEQ ID NO: 6 - DNA, 45 bp, Artificial Sequence
  CK1 Light Chain CDR3
tattattgtcagcagagtagcgccatcccttataccttcggtcag

SEQ ID NO: 7 - protein, 12 aa, Artificial Sequence
  CK1 Heavy Chain CDR1
FTFSRYAMTWVR

SEQ ID NO: 8 - protein, 13 aa, Artificial Sequence
  CK1 Heavy Chain CDR2
SMSGTGGTTYYAD

SEQ ID NO: 9 - protein, 12 aa, Artificial Sequence
  CK1 Heavy Chain CDR3
YCARGAYGFDHW

SEQ ID NO: 10 - protein, 13 aa, Artificial Sequence
  CK1 Light Chain CDR1
CRASQSIGNYLNW

SEQ ID NO: 11 - protein, 10 aa, Artificial Sequence
  CK1 Light Chain CDR2
DASNLETGIP

SEQ ID NO: 12 - protein, 12 aa, Artificial Sequence
  CK1 Light Chain CDR3
YCQQSSAIPYTF

SEQ ID NO: 13 - DNA, 30 bp, Artificial Sequence
  CK2 Heavy Chain CDR1
ttcagcagctatggcatgcattgggttcgc

SEQ ID NO: 14 - DNA, 45 bp, Artificial Sequence
  CK2 Heavy Chain CDR2
agcgccatcagcggcagcggcaccagcatctattatgccgatagc

SEQ ID NO: 15 - DNA, 36 bp, Artificial Sequence
  CK2 Heavy Chain CDR3
tactgtgcccgcggcggcaccgcctttgattattgg

SEQ ID NO: 16 - DNA, 39 bp, Artificial Sequence
  CK2 Light Chain CDR1
tgccgcgccagccagagatcagacaactatctggcctgg

SEQ ID NO: 17 - DNA, 36 bp, Artificial Sequence
  CK2 Light Chain CDR2
ctgatctatgatgccagcaaccgcgccaccggcatc

SEQ ID NO: 18 - DNA, 45 bp, Artificial Sequence
  CK2 Light Chain CDR3
tattattgtcagcagagctatagcaccccttttaccttcggtcag

SEQ ID NO: 19 - protein, 12 aa, Artificial Sequence
  CK2 Heavy Chain CDR1
FTFSSYGMHWVR

SEQ ID NO: 20 - protein, 13 aa, Artificial Sequence
  CK2 Heavy Chain CDR2
AISGSGTSIYYAD

SEQ ID NO: 21 - protein, 12 aa, Artificial Sequence
  CK2 Heavy Chain CDR3
YCARGGTAFDYW

SEQ ID NO: 22 - protein, 13 aa, Artificial Sequence
  CK2 Light Chain CDR1
CRASQRSDNYLAW

SEQ ID NO: 23 - protein, 10 aa, Artificial Sequence
  CK2 Light Chain CDR2
DASNRATGIP

SEQ ID NO: 24 - protein, 12 aa, Artificial Sequence
  CK2 Light Chain CDR3
YCQQSYSTPFTF

SEQ ID NO: 25 - DNA, 30 bp, Artificial Sequence
  CK3 Heavy Chain CDR1
ttcagcagctatgccatcagctgggttcgc

SEQ ID NO: 26 - DNA, 45 bp, Artificial Sequence
  CK3 Heavy Chain CDR2
agcgccaccagcggcagcggccgcgccacctattatgccgatagc

SEQ ID NO: 27 - DNA, 45 bp, Artificial Sequence
  CK3 Heavy Chain CDR3
tactgtgcgcgcgatacctggtgggaaggctattttgatctgtgg

SEQ ID NO: 28 - DNA, 36 bp, Artificial Sequence
  CK3 Light Chain CDR1
tgccaggccagccatatcagcacccatctgaactgg

SEQ ID NO: 29 - DNA, 36 bp, Artificial Sequence
  CK3 Light Chain CDR2
ctgatctatggcgccagcagccgcgccaccggcatc

SEQ ID NO: 30 - DNA, 45 bp, Artificial Sequence
  CK3 Light Chain CDR3
tattattgtcagcagtataacacctatcctcctaccttcggtcag

SEQ ID NO: 31 - protein, 12 aa, Artificial Sequence
  CK3 Heavy Chain CDR1
FTFSSYAISWVR

SEQ ID NO: 32 - protein, 13 aa, Artificial Sequence
  CK3 Heavy Chain CDR2
ATSGSGRATYYAD

SEQ ID NO: 33 - protein, 15 aa, Artificial Sequence
  CK3 Heavy Chain CDR3
YCARDTWWEGYFDLW

SEQ ID NO: 34 - protein, 12 aa, Artificial Sequence
  CK3 Light Chain CDR1
CQASHISTHLNW

SEQ ID NO: 35 - protein, 10 aa, Artificial Sequence
  CK3 Light Chain CDR2
GASSRATGIP

SEQ ID NO: 36 - protein, 12 aa, Artificial Sequence
  CK3 Light Chain CDR3
YCQQYNTYPPTF

SEQ ID NO: 37 - DNA, 33 bp, Artificial Sequence
  CL4 Heavy Chain CDR1
accttcggcagcaactatatgagctgggttcgc

SEQ ID NO: 38 - DNA, 33 bp, Artificial Sequence
  CL4 Heavy Chain CDR2
atcagcggcagcggcaccagcacctattatgcc

SEQ ID NO: 39 - DNA, 27 bp, Artificial Sequence
  CL4 Heavy Chain CDR3
cgcggcatgtggggcatggatgtgtgg

SEQ ID NO: 40 - DNA, 27 bp, Artificial Sequence
  CL4 Light Chain CDR1
ggcaaacatcggcacaccgtgaactgg

SEQ ID NO: 41 - DNA, 30 bp, Artificial Sequence
  CL4 Light Chain CDR2
ctggatagcgaacgccctagcggcgtacct

SEQ ID NO: 42 - DNA, 27 bp, Artificial Sequence
  CL4 Light Chain CDR3
tatgatagcagcagcgtggtgtttggt

SEQ ID NO: 43 - protein, 12 aa, Artificial Sequence
  CL4 Heavy Chain CDR1
FTFGSNYMSWVR

SEQ ID NO: 44 - protein, 13 aa, Artificial Sequence
  CL4 Heavy Chain CDR2
TISGSGTSTYYAD

SEQ ID NO: 45 - protein, 12 aa, Artificial Sequence
  CL4 Heavy Chain CDR3
YCARGMWGMDVW

SEQ ID NO: 46 - protein, 11 aa, Artificial Sequence
  CL4 Light Chain CDR1
CTGKHRHTVNW

SEQ ID NO: 47 - protein, 10 aa, Artificial Sequence
  CL4 Light Chain CDR2
LDSERPSGVP

SEQ ID NO: 48 - protein, 12 aa, Artificial Sequence
  CL4 Light Chain CDR3
YCQSYDSSSVVF

SEQ ID NO: 49 - DNA, 33 bp, Artificial Sequence
  CL5 Heavy Chain CDR1
accttcagcagctatgccatgcattgggttcgc

SEQ ID NO: 50 - DNA, 33 bp, Artificial Sequence
  CL5 Heavy Chain CDR2
atcagcggcggcggctatggcacctattatgcc

SEQ ID NO: 51 - DNA, 30 bp, Artificial Sequence
  CL5 Heavy Chain CDR3
cgcagcaccgtgtgggcctttgatatctgg

SEQ ID NO: 52 - DNA, 30 bp, Artificial Sequence
  CL5 Light Chain CDR1
ggcaacaacatcggcagcaaaagcgtgcat

SEQ ID NO: 53 - DNA, 30 bp, Artificial Sequence
  CL5 Light Chain CDR2
gatgtgagcaaacgccctagcgagcgtcct

SEQ ID NO: 54 - DNA, 30 bp, Artificial Sequence
  CL5 Light Chain CDR3
tttgatagcagcggcacctggatctttggt

SEQ ID NO: 55 - protein, 12 aa, Artificial Sequence
  CL5 Heavy Chain CDR1
FTFSSYAMHWVR

SEQ ID NO: 56 - protein, 13 aa, Artificial Sequence
  CL5 Heavy Chain CDR2
SISGGGYGTYYAD

SEQ ID NO: 57 - protein, 13 aa, Artificial Sequence
  CL5 Heavy Chain CDR3
YCARSTVWAFDIW

SEQ ID NO: 58 - protein, 13 aa, Artificial Sequence
  CL5 Light Chain CDR1
CSGNNIGSKSVHW

SEQ ID NO: 59 - protein, 11 aa, Artificial Sequence
  CL5 Light Chain CDR2
DVSKRPSERPD

SEQ ID NO: 60 - protein, 13 aa, Artificial Sequence
  CL5 Light Chain CDR3
YCQSFDSSGTWIF

SEQ ID NO: 61 - DNA, 27 bp, Artificial Sequence
  CL6 Heavy Chain CDR1
agcagctacggtatgcattgggtcaga

SEQ ID NO: 62 - DNA, 39 bp, Artificial Sequence
  CL6 Heavy Chain CDR2
gcaattagcggtagcggtggtagcacttactacgcagac

SEQ ID NO: 63 - DNA, 45 bp, Artificial Sequence
  CL6 Heavy Chain CDR3
tgcgcagtcagtggtgcaggtcgtggtttcttcgactactgggga

SEQ ID NO: 64 - DNA, 39 bp, Artificial Sequence
  CL6 Light Chain CDR1
tgcagcggtagcagcagcaacattggtagcaactacgtg

SEQ ID NO: 65 - DNA, 24 bp, Artificial Sequence
  CL6 Light Chain CDR2
gacaacaagcgtcctagtggtgtg

SEQ ID NO: 66 - DNA, 33 bp, Artificial Sequence
  CL6 Light Chain CDR3
tgcagcagctacactagcagcagcactgtgatc

SEQ ID NO: 67 - protein, 12 aa, Artificial Sequence
  CL6 Heavy Chain CDR1
FTFSSYGMHWVR

SEQ ID NO: 68 - protein, 13 aa, Artificial Sequence
  CL6 Heavy Chain CDR2
AISGSGGSTYYAD

SEQ ID NO: 69 - protein, 15 aa, Artificial Sequence
  CL6 Heavy Chain CDR3
YCAVSGAGRGFFDYW

SEQ ID NO: 70 - protein, 15 aa, Artificial Sequence
  CL6 Light Chain CDR1
CSGSSSNIGSNYVYW

SEQ ID NO: 71 - protein, 10 aa, Artificial Sequence
  CL6 Light Chain CDR2
EDNKRPSGVP

SEQ ID NO: 72 - protein, 13 aa, Artificial Sequence
  CL6 Light Chain CDR3
YCSSYTSSSTVIF

SEQ ID NO: 73 - DNA, 27 bp, Artificial Sequence
  CL7 Heavy Chain CDR1
agccgctacgcaatgagctgggtcaga

SEQ ID NO: 74 - DNA, 39 bp, Artificial Sequence; identical to SEQ ID NO: 62
  CL7 Heavy Chain CDR2

SEQ ID NO: 75 - DNA, 39 bp, Artificial Sequence
  CL7 Heavy Chain CDR3
tgcgcacgtagcagccagggtatcttcgacatctgggga

SEQ ID NO: 76 - DNA, 33 bp, Artificial Sequence
  CL7 Light Chain CDR1
tgcagtggtaacaatatcggtactagacgcgtg

SEQ ID NO: 77 - DNA, 24 bp, Artificial Sequence
  CL7 Light Chain CDR2
aagaacaaccgtcctagtggtgtg

SEQ ID NO: 78 - DNA, 39 bp, Artificial Sequence
  CL7 Light Chain CDR3
tgcgcagcatgggacgacagcctgagcggtcctgtgttc

SEQ ID NO: 79 - protein, 12 aa, Artificial Sequence
  CL7 Heavy Chain CDR1
FTFSRYAMSWVR

SEQ ID NO: 80 - protein, 13 aa, Artificial Sequence
  CL7 Heavy Chain CDR2
AISGSGGSTYYAD

SEQ ID NO: 81 - protein, 13 aa, Artificial Sequence
  CL7 Heavy Chain CDR3
YCARSSQGIFDIW

SEQ ID NO: 82 - protein, 13 aa, Artificial Sequence
  CL7 Light Chain CDR1
CSGNNIGTRRVHW

SEQ ID NO: 83 - protein, 10 aa, Artificial Sequence
  CL7 Light Chain CDR2
SKNNRPSGVP

SEQ ID NO: 84 - protein, 14 aa, Artificial Sequence
  CL7 Light Chain CDR3
YCAAWDDSLSGPVF

SEQ ID NO: 85 - DNA, 27 bp, Artificial Sequence
  CL8 Heavy Chain CDR1
agcagctacgcaatgagctgggtcaga

SEQ ID NO: 86 - DNA, 39 bp, Artificial Sequence; identical to SEQ ID NO: 62
  CL8 Heavy Chain CDR2

SEQ ID NO: 87 - DNA, 42 bp, Artificial Sequence
  CL8 Heavy Chain CDR3
tgcgcacgtagcggtcgttacgcagacttgacatctggggga

SEQ ID NO: 88 - DNA, 39 bp, Artificial Sequence
  CL8 Light Chain CDR1
tgcagcggtagcaacagcaacatcggtaacaactacgtg

SEQ ID NO: 89 - DNA, 24 bp, Artificial Sequence
  CL8 Light Chain CDR2
aacaacaagcgtcctagtggtgtg

SEQ ID NO: 90 - DNA, 36 bp, Artificial Sequence
  CL8 Light Chain CDR3
tgcagcagctacactagcagcagcactgtgatgttc

SEQ ID NO: 91 - protein, 12 aa, Artificial Sequence
  CL8 Heavy Chain CDR1
FTFSSYAMSWVR

SEQ ID NO: 92 - protein, 13 aa, Artificial Sequence
  CL8 Heavy Chain CDR2
AISGSGGSTYYAD

SEQ ID NO: 93 - protein, 14 aa, Artificial Sequence
  CL8 Heavy Chain CDR3
YCARSGRYADLTSG

SEQ ID NO: 94 - protein, 15 aa, Artificial Sequence
  CL8 Light Chain CDR1
CSGSNSNIGNNYVSW

SEQ ID NO: 95 - protein, 10 aa, Artificial Sequence
  CL8 Light Chain CDR2
DNNKRPSGVP

SEQ ID NO: 96 - protein, 13 aa, Artificial Sequence
  CL8 Light Chain CDR3
YCSSYTSSSTVMF

SEQ ID NO: 97 - DNA, 27 bp, Artificial Sequence
  CL9 Heavy Chain CDR1
agcagctactactggagctgggtcaga

SEQ ID NO: 98 - DNA, 39 bp, Artificial Sequence; identical to SEQ ID NO: 62
  CL9 Heavy Chain CDR2

SEQ ID NO: 99 - DNA, 39 bp, Artificial Sequence
  CL9 Heavy Chain CDR3
tgcgcacgtatcgacgtgtacggtttcgacatctgggga

SEQ ID NO: 100 - DNA, 39 bp, Artificial Sequence
  CL9 Light Chain CDR1
tgcagcggtagcactagcaacatcggtactaactacgtg

SEQ ID NO: 101 - DNA, 24 bp, Artificial Sequence
  CL9 Light Chain CDR2
aacaacaaccgtcctagtggtgtg

SEQ ID NO: 102 - DNA, 33 bp, Artificial Sequence
  CL9 Light Chain CDR3
tgccagacttgggacagcagcactgacgtagtg

SEQ ID NO: 103 - protein, 12 aa, Artificial Sequence
  CL9 Heavy Chain CDR1
FTFSSYYWSWVR

SEQ ID NO: 104 - protein, 13 aa, Artificial Sequence
  CL9 Heavy Chain CDR2
AISGSGGSTYYAD

SEQ ID NO: 105 - protein, 13 aa, Artificial Sequence
  CL9 Heavy Chain CDR3
YCARIDVYGFDIW

SEQ ID NO: 106 - protein, 15 aa, Artificial Sequence
  CL9 Light Chain CDR1
CSGSTSNIGTNYVYW

SEQ ID NO: 107 - protein, 10 aa, Artificial Sequence
  CL9 Light Chain CDR2
DNNNRPSGVP

SEQ ID NO: 108 - protein, 13 aa, Artificial Sequence
  CL9 Light Chain CDR3
YCQTWDSSTDVVF

SEQ ID NO: 109 - DNA, 31 bp, Artificial Sequence
  CL10 Heavy Chain CDR1
tcagcagctacggtatgcattgggtcagaca

SEQ ID NO: 110 - DNA, 43 bp, Artificial Sequence
  CL10 Heavy Chain CDR2
ctgcaattagcggtagcggtggtagcacttactacgcagacag

SEQ ID NO: 111 - DNA, 40 bp, Artificial Sequence
  CL10 Heavy Chain CDR3
actgcgcaagcggttacggtctgatggacgtgtggggaca

SEQ ID NO: 112 - DNA, 43 bp, Artificial Sequence
  CL10 Light Chain CDR1
gctgcactcgtagcagcggtatcatcgcaagcaactacgtgca

SEQ ID NO: 113 - DNA, 27 bp, Artificial Sequence
  CL10 Light Chain CDR2
cgcaacaaccagcgccctagtggtgtg

SEQ ID NO: 114 - DNA, 40 bp, Artificial Sequence
  CL10 Light Chain CDR3
actgcagcagctacgcaggtaacaacaacctggtgttcgg

SEQ ID NO: 115 - protein, 12 aa, Artificial Sequence
  CL10 Heavy Chain CDR1
FTFSSYGMHWVR

SEQ ID NO: 116 - protein, 13 aa, Artificial Sequence
  CL10 Heavy Chain CDR2
AISGSGGSTYYAD

SEQ ID NO: 117 - protein, 12 aa, Artificial Sequence
  CL10 Heavy Chain CDR3
YCASGYGLMDVW

SEQ ID NO: 118 - protein, 15 aa, Artificial Sequence
  CL10 Light Chain CDR1
CTRSSGIIASNYVQW

SEQ ID NO: 119 - protein, 10 aa, Artificial Sequence
  CL10 Light Chain CDR2
RNNQRPSGVP

SEQ ID NO: 120 - protein, 13 aa, Artificial Sequence
  CL10 Light Chain CDR3
YCSSYAGNNNLVF

SEQ ID NO: 121 - DNA, 30 bp, Artificial Sequence
  SK11 Heavy Chain CDR1
ttcagcacctatggcatgcattgggttcgc

SEQ ID NO: 122 - DNA, 42 bp, Artificial Sequence
  SK11 Heavy Chain CDR2
agcgccatcagcggcagcggcggcagcacctattatgccgat

SEQ ID NO: 123 - DNA, 36 bp, Artificial Sequence
  SK11 Heavy Chain CDR3
tactgtgcccgcggcctgagcggccttgattattgg

SEQ ID NO: 124 - DNA, 39 bp, Artificial Sequence
  SK11 Light Chain CDR1
tgccgctccagccagggcatcaccaactatctggcctgg

SEQ ID NO: 125 - DNA, 36 bp, Artificial Sequence; identical to SEQ ID NO: 17
  SK11 Light Chain CDR2

SEQ ID NO: 126 - DNA, 45 bp, Artificial Sequence
  SK11 Light Chain CDR3
tattattgtcagcagagctatagcacccctctgaccttcggtcag

SEQ ID NO: 127 - protein, 12 aa, Artificial Sequence
  SK11 Heavy Chain CDR1
FTFSTYGMHWVR

SEQ ID NO: 128 - protein, 13 aa, Artificial Sequence
  SK11 Heavy Chain CDR2
AISGSGGSTYYAD

SEQ ID NO: 129 - protein, 12 aa, Artificial Sequence
  SK11 Heavy Chain CDR3
YCARGLSGLDYW

SEQ ID NO: 130 - protein, 13 aa, Artificial Sequence
  SK11 Light Chain CDR1
CRSSQGITNYLAW

SEQ ID NO: 131 - protein, 10 aa, Artificial Sequence
  SK11 Light Chain CDR2
DASNRATGIP

SEQ ID NO: 132 - protein, 12 aa, Artificial Sequence
  SK11 Light Chain CDR3
YCQQSYSTPLTF

SEQ ID NO: 133 - DNA, 34 bp, Artificial Sequence
  SK12 Heavy Chain CDR1
ccttcagcagctatgccatgcattgggttcgcca

SEQ ID NO: 134 - DNA, 49 bp, Artificial Sequence
  SK12 Heavy Chain CDR2
tgagcgccatcagcggcagcggcggcgatacctatcatgccgatagcgt

SEQ ID NO: 135 - DNA, 40 bp, Artificial Sequence
  SK12 Heavy Chain CDR3
actactgtacccgcggcctgagcggctttgattattgggg

SEQ ID NO: 136 - DNA, 43 bp, Artificial Sequence
  SK12 Light Chain CDR1
catgccgcgccagccagagcatcagcagctatctgaactggta

SEQ ID NO: 137 - DNA, 40 bp, Artificial Sequence
  SK12 Light Chain CDR2
tgctgatctatgatgccagcaaccgcgcccctggcatccc

SEQ ID NO: 138 - DNA, 49 bp, Artificial Sequence
  SK12 Light Chain CDR3
tgtattattgtcagcagagctatagcatccctatcaccttcggtcaggg

SEQ ID NO: 139 - protein, 12 aa, Artificial Sequence
  SK12 Heavy Chain CDR1
FTFSSYAMHWVR

SEQ ID NO: 140 - protein, 13 aa, Artificial Sequence
  SK12 Heavy Chain CDR2
AISGSGGDTYHAD

SEQ ID NO: 141 - protein, 12 aa, Artificial Sequence
  SK12 Heavy Chain CDR3
YCTRGLSGFDYW

SEQ ID NO: 142 - protein, 13 aa, Artificial Sequence
  SK12 Light Chain CDR1
CRASQSISSYLNW

SEQ ID NO: 143 - protein, 10 aa, Artificial Sequence
  SK12 Light Chain CDR2
DASNRAPGIP

SEQ ID NO: 144 - protein, 12 aa, Artificial Sequence
  SK12 Light Chain CDR3
YCQQSYSIPITF

SEQ ID NO: 145 - DNA, 30 bp, Artificial Sequence
  SK13 Heavy Chain CDR1
ttcagcgattatgccatgagctgggttcgc

SEQ ID NO: 146 - DNA, 42 bp, Artificial Sequence
  SK13 Heavy Chain CDR2
agcatcagcagcagcagcagctatatctactataccgatagc

SEQ ID NO: 147 - DNA, 36 bp, Artificial Sequence
  SK13 Heavy Chain CDR3
tactgtgcccgcggcggctatggctttgattattgg

SEQ ID NO: 148 - DNA, 39 bp, Artificial Sequence
  SK13 Light Chain CDR1
tgccgcgccagccagagcatcagcagctatctgaactgg

SEQ ID NO: 149 - DNA, 36 bp, Artificial Sequence
  SK13 Light Chain CDR2
ctgatctatagcgccagcagccgcccacagggcatc

SEQ ID NO: 150 - DNA, 45 bp, Artificial Sequence
  SK13 Light Chain CDR3
tattattgtcagcagtatgatgatctgccttttaccttcggtcag

SEQ ID NO: 151 - protein, 12 aa, Artificial Sequence
  SK13 Heavy Chain CDR1
FTFSDYAMSWVR

SEQ ID NO: 152 - protein, 13 aa, Artificial Sequence
  SK13 Heavy Chain CDR2
SISSSSSYIYYTD

SEQ ID NO: 153 - protein, 12 aa, Artificial Sequence
  SK13 Heavy Chain CDR3
YCARGGYGFDYW

SEQ ID NO: 154 - protein, 13 aa, Artificial Sequence
  SK13 Light Chain CDR1
CRASQSISSYLNW

SEQ ID NO: 155 - protein, 10 aa, Artificial Sequence
  SK13 Light Chain CDR2
SASSRPQGIP

SEQ ID NO: 156 - protein, 12 aa, Artificial Sequence
  SK13 Light Chain CDR3
YCQQYDDLPFTF

SEQ ID NO: 157 - DNA, 34 bp, Artificial Sequence
  SK14 Heavy Chain CDR1
ccttcagcaactttgcgatcgcctgggttcgcca

SEQ ID NO: 158 - DNA, 46 bp, Artificial Sequence
  SK14 Heavy Chain CDR2
gcgccatcagcggccgcggcaccagcacctattatgccgatagcgt

SEQ ID NO: 159 - DNA, 40 bp, Artificial Sequence
  SK14 Heavy Chain CDR3
actactgtgcccgcggcgtgagcggctttgatagctgggg

SEQ ID NO: 160 - DNA, 43 bp, Artificial Sequence
  SK14 Light Chain CDR1
catgccgcgccagccagagcatcagcagccatctggcctggta

SEQ ID NO: 161 - DNA, 40 bp, Artificial Sequence
  SK14 Light Chain CDR2
tgctgatctatgataccagcaaccgcgccaccggcatccc

SEQ ID NO: 162 - DNA, 49 bp, Artificial Sequence
  SK14 Light Chain CDR3
tgtactattgtcagcagagctatagcaccccttttaccttcggtcaggg

SEQ ID NO: 163 - protein, 12 aa, Artificial Sequence
  SK14 Heavy Chain CDR1
FTFSNFAIAWVR

SEQ ID NO: 164 - protein, 13 aa, Artificial Sequence
  SK14 Heavy Chain CDR2
AISGRGTSTYYAD

SEQ ID NO: 165 - protein, 12 aa, Artificial Sequence
  SK14 Heavy Chain CDR3
YCARGVSGFDSW

SEQ ID NO: 166 - protein, 13 aa, Artificial Sequence
  SK14 Light Chain CDR1
CRASQSISSHLAW

SEQ ID NO: 167 - protein, 10 aa, Artificial Sequence
  SK14 Light Chain CDR2
DTSNRATGIP

SEQ ID NO: 168 - protein, 12 aa, Artificial Sequence
  SK14 Light Chain CDR3
YCQQSYSTPFTF

SEQ ID NO: 169 - DNA, 34 bp, Artificial Sequence; identical to SEQ ID NO: 133
  SK15 Heavy Chain CDR1

SEQ ID NO: 170 - DNA, 49 bp, Artificial Sequence
  SK15 Heavy Chain CDR2
tgagcgccatcaacggcagcggcggcagcacctattatgccgatagcgt

SEQ ID NO: 171 - DNA, 43 bp, Artificial Sequence
  SK15 Heavy Chain CDR3
actactgtgcccgcggcctgcagggctttgattattggggaca

SEQ ID NO: 172 - DNA, 43 bp, Artificial Sequence
  SK15 Light Chain CDR1
catgccaggccagccaggatatcaccaactatctgaactggta

SEQ ID NO: 173 - DNA, 40 bp, Artificial Sequence
  SK15 Light Chain CDR2
tgctgatctatgatgccagcagcctggaaaccggcatccc

SEQ ID NO: 174 - DNA, 49 bp, Artificial Sequence
  SK15 Light Chain CDR3
tgtattattgtcagcagagctatagcacccctatcaccttcggtcaggg

SEQ ID NO: 175 - protein, 12 aa, Artificial Sequence
  SK15 Heavy Chain CDR1
FTFSSYAMHWVR

SEQ ID NO: 176 - protein, 13 aa, Artificial Sequence
  SK15 Heavy Chain CDR2
AINGSGGSTYYAD

SEQ ID NO: 177 - protein, 12 aa, Artificial Sequence
  SK15 Heavy Chain CDR3
YCARGLQGFDYW

SEQ ID NO: 178 - protein, 13 aa, Artificial Sequence
  SK15 Light Chain CDR1
CQASQDITNYLNW

SEQ ID NO: 179 - protein, 10 aa, Artificial Sequence
  SK15 Light Chain CDR2
DASSLETGIP

SEQ ID NO: 180 - protein, 12 aa, Artificial Sequence
  SK15 Light Chain CDR3
YCQQSYSTPITF

SEQ ID NO: 181 - DNA, 34 bp, Artificial Sequence
  SK16 Heavy Chain CDR1
ccttcagcagctatgccatgagctgggttcgcca

SEQ ID NO: 182 - DNA, 49 bp, Artificial Sequence
  SK16 Heavy Chain CDR2
tgagcgccatcaacggcagcggcggcagcaccctgtatgccgatagcgt

SEQ ID NO: 183 - DNA, 40 bp, Artificial Sequence; identical to SEQ ID NO: 159
  SK16 Heavy Chain CDR3

SEQ ID NO: 184 - DNA, 43 bp, Artificial Sequence
  SK16 Light Chain CDR1
catgccgcatcagccagagcatcagcagctatctgaactggta

SEQ ID NO: 185 - DNA, 40 bp, Artificial Sequence
  SK16 Light Chain CDR2
tgctgatctatgatgccagcctgcgcgccaccggcatccc

SEQ ID NO: 186 - DNA, 49 bp, Artificial Sequence
  SK16 Light Chain CDR3
tgtattattgtcagcagagctataaaacccctatcaccttcggtcaggg

SEQ ID NO: 187 - protein, 12 aa, Artificial Sequence
  SK16 Heavy Chain CDR1
FTFSSYAMSWVR

SEQ ID NO: 188 - protein, 13 aa, Artificial Sequence
  SK16 Heavy Chain CDR2
AINGSGGSTLYAD

SEQ ID NO: 189 - protein, 12 aa, Artificial Sequence
  SK16 Heavy Chain CDR3
YCARGVSGFDSW

SEQ ID NO: 190 - protein, 13 aa, Artificial Sequence
  SK16 Light Chain CDR1
CRISQSISSYLNW

SEQ ID NO: 191 - protein, 10 aa, Artificial Sequence
  SK16 Light Chain CDR2
DASLRATGIP

SEQ ID NO: 192 - protein, 13 aa, Artificial Sequence
  SK16 Light Chain CDR3
YYCQQSYKTPITF

SEQ ID NO: 193 - DNA, 34 bp, Artificial Sequence
  SK17 Heavy Chain CDR1
ccttcagcagctattattggagctgggttcgcca

SEQ ID NO: 194 - DNA, 49 bp, Artificial Sequence
  SK17 Heavy Chain CDR2
tgagcaccatcaccggcagcggcggcagcaccgattatgccaacagcgt

SEQ ID NO: 195 - DNA, 40 bp, Artificial Sequence
  SK17 Heavy Chain CDR3
actactgtgccaccggcggcggcatctttgactattgggg

SEQ ID NO: 196 - DNA, 43 bp, Artificial Sequence
  SK17 Light Chain CDR1
catgccaggccagccagaccatcagcaactatctgaactggta

SEQ ID NO: 197 - DNA, 40 bp, Artificial Sequence
  SK17 Light Chain CDR2
tgctgatctatgatgccagcaaccgcgccaccggcatccc

SEQ ID NO: 198 - DNA, 49 bp, Artificial Sequence
  SK17 Light Chain CDR3
tgtattattgtcagcagtacaacagctatcctcctagcttcggtcaggg

SEQ ID NO: 199 - protein, 12 aa, Artificial Sequence
  SK17 Heavy Chain CDR1
FTFSSYYWSWVR

SEQ ID NO: 200 - protein, 13 aa, Artificial Sequence
  SK17 Heavy Chain CDR2
TITGSGGSTDYAN

SEQ ID NO: 201 - protein, 12 aa, Artificial Sequence
  SK17 Heavy Chain CDR3
YCATGGGIFDYW

SEQ ID NO: 202 - protein, 13 aa, Artificial Sequence
  SK17 Light Chain CDR1
CQASQTISNYLNW

SEQ ID NO: 203 - protein, 10 aa, Artificial Sequence
  SK17 Light Chain CDR2
DASNRATGIP

SEQ ID NO: 204 - protein, 12 aa, Artificial Sequence
  SK17 Light Chain CDR3
YCQQYNSYPPSF

SEQ ID NO: 205 - DNA, 34 bp, Artificial Sequence
  SL18 Heavy Chain CDR1
tcaccttcagcgattatcatatgcattgggttcg

SEQ ID NO: 206 - DNA, 34 bp, Artificial Sequence
  SL18 Heavy Chain CDR2
tcagcagcagcggcggctatacctattatgccga

SEQ ID NO: 207 - DNA, 34 bp, Artificial Sequence
  SL18 Heavy Chain CDR3
cccgatcgatacgcctgcctctggattattgggg

SEQ ID NO: 208 - DNA, 37 bp, Artificial Sequence
  SL18 Light Chain CDR1
gcggcaacaacatcggcagcaaaggcgtgcattggta

SEQ ID NO: 209 - DNA, 34 bp, Artificial Sequence
  SL18 Light Chain CDR2
atgaagatagcaaacgccctagcggcgtgcgtga

SEQ ID NO: 210 - DNA, 34 bp, Artificial Sequence
  SL18 Light Chain CDR3
gctatgatagcaccaaaggcgtggtgtttggtgg

SEQ ID NO: 211 - protein, 12 aa, Artificial Sequence
  SL18 Heavy Chain CDR1
FTFSDYHMHWVR

SEQ ID NO: 212 - protein, 13 aa, Artificial Sequence
  SL18 Heavy Chain CDR2
TISSSGGYTYYAE

SEQ ID NO: 213 - protein, 13 aa, Artificial Sequence
  SL18 Heavy Chain CDR3
YCARSIRLPLDYW

SEQ ID NO: 214 - protein, 13 aa, Artificial Sequence
  SL18 Light Chain CDR1
CSGNNIGSKGVHW

SEQ ID NO: 215 - protein, 10 aa, Artificial Sequence
  SL18 Light Chain CDR2
EDSKRPSGVR

SEQ ID NO: 216 - protein, 13 aa, Artificial Sequence
  SL18 Light Chain CDR3
YCQSYDSTKGVVF

SEQ ID NO: 217 - DNA, 34 bp, Artificial Sequence
  CB301_H3L1_A10 Heavy Chain CDR1
tcagcagctacggtatgcattgggtcagacaggc

SEQ ID NO: 218 - DNA, 43 bp, Artificial Sequence; identical to SEQ ID NO: 110
  CB301_H3L1_A10 Heavy Chain CDR2

SEQ ID NO: 219 - DNA, 40 bp, Artificial Sequence
  CB301_H3L1_A10 Heavy Chain CDR3
actgcgtgcgtggttacggtgcaatggacgtgtggggaca

SEQ ID NO: 220 - DNA, 43 bp, Artificial Sequence
  CB301_H3L1_A10 Light Chain CDR1
gctgcactcgtagcagcggtagcatcgcaagcaactacgtgca

SEQ ID NO: 221 - DNA, 31 bp, Artificial Sequence
  CB301_H3L1_A10 Light Chain CDR2
accgcaacaaccagcgccctagtggtgtgcc

SEQ ID NO: 222 - DNA, 40 bp, Artificial Sequence
  CB301_H3L1_A10 Light Chain CDR3
actgcagcagctacactactagcagcactctggtgttcgg

SEQ ID NO: 223 - protein, 12 aa, Artificial Sequence
  CB301_H3L1_A10 Heavy Chain CDR1
FTFSSYGMHWVR

SEQ ID NO: 224 - protein, 13 aa, Artificial Sequence
  CB301_H3L1_A10 Heavy Chain CDR2
AISGSGGSTYYAD

SEQ ID NO: 225 - protein, 12 aa, Artificial Sequence
  CB301_H3L1_A10 Heavy Chain CDR3
YCVRGYGAMDVW

SEQ ID NO: 226 - protein, 15 aa, Artificial Sequence
  CB301_H3L1_A10 Light Chain CDR1
CTRSSGSIASNYVQW

SEQ ID NO: 227 - protein, 10 aa, Artificial Sequence
  CB301_H3L1_A10 Light Chain CDR2
RNNQRPSGVP

SEQ ID NO: 228 - protein, 13 aa, Artificial Sequence
  CB301_H3L1_A10 Light Chain CDR3
YCSSYTTSSTLVF

SEQ ID NO: 229 - DNA, 34 bp, Artificial Sequence
  CB301_H3L1_A12 Heavy Chain CDR1
tcagcagctacgcaatgcattgggtcagacaggc

SEQ ID NO: 230 - DNA, 43 bp, Artificial Sequence; identical to SEQ ID NO: 110
  CB301_H3L1_A12 Heavy Chain CDR2

SEQ ID NO: 231 - DNA, 40 bp, Artificial Sequence
  CB301_H3L1_A12 Heavy Chain CDR3
actgcgcaagcggctacggtctgatggacgtatggggaca

SEQ ID NO: 232 - DNA, 46 bp, Artificial Sequence
  CB301_H3L1_A12 Light Chain CDR1
gctgcactggtactagcagcgacgtgggtaactacaacctggtgag

SEQ ID NO: 233 - DNA, 31 bp, Artificial Sequence
  CB301_H3L1_A12 Light Chain CDR2
acagcaacaaccagcgccctagtggtgtgcc

SEQ ID NO: 234 - DNA, 40 bp, Artificial Sequence
  CB301_H3L1_A12 Light Chain CDR3
actgcagcagctacactggtagcaacgctctgttgttcgg

SEQ ID NO: 235 - protein, 12 aa, Artificial Sequence
  CB301_H3L1_A12 Heavy Chain CDR1
FTFSSYAMHWVR

SEQ ID NO: 236 - protein, 13 aa, Artificial Sequence
  CB301_H3L1_A12 Heavy Chain CDR2
AISGSGGSTYYAD

SEQ ID NO: 237 - protein, 12 aa, Artificial Sequence
  CB301_H3L1_A12 Heavy Chain CDR3
YCASGYGLMDVW

SEQ ID NO: 238 - protein, 16 aa, Artificial Sequence
  CB301_H3L1_A12 Light Chain CDR1
CTGTSSDVGNYNLVSW

SEQ ID NO: 239 - protein, 10 aa, Artificial Sequence
  CB301_H3L1_A12 Light Chain CDR2
SNNQRPSGVP

SEQ ID NO: 240 - protein, 13 aa, Artificial Sequence
  CB301_H3L1_A12 Light Chain CDR3
YCSSYTGSNALLF

SEQ ID NO: 241 - DNA, 31 bp, Artificial Sequence
  CB301_H3L1_E6 Heavy Chain CDR1
tcagcagctacgcaatgagctgggtcagaca

SEQ ID NO: 242 - DNA, 43 bp, Artificial Sequence; identical to SEQ ID NO: 110
  CB301_H3L1_E6 Heavy Chain CDR2

SEQ ID NO: 243 - DNA, 40 bp, Artificial Sequence
  CB301_H3L1_E6 Heavy Chain CDR3
actgcgcacgctggcattacagcttcgactactggggaca

SEQ ID NO: 244 - DNA, 37 bp, Artificial Sequence
  CB301_H3L1_E6 Light Chain CDR1
gctgccgtggtaacaacatcggtagcaagcgtgtgca

SEQ ID NO: 245 - DNA, 31 bp, Artificial Sequence
  CB301_H3L1_E6 Light Chain CDR2
acagctacaaccaccgtcctagcggtgtgcc

SEQ ID NO: 246 - DNA, 43 bp, Artificial Sequence
  CB301_H3L1_E6 Light Chain CDR3
actgcaacacttgggacgacagcctggagggtcctgtgttcgg

SEQ ID NO: 247 - protein, 12 aa, Artificial Sequence
  CB301_H3L1_E6 Heavy Chain CDR1
FTFSSYAMSWVR

SEQ ID NO: 248 - protein, 13 aa, Artificial Sequence
  CB301_H3L1_E6 Heavy Chain CDR2
AISGSGGSTYYAD

SEQ ID NO: 249 - protein, 12 aa, Artificial Sequence
  CB301_H3L1_E6 Heavy Chain CDR3
YCARWHYSFDYW

SEQ ID NO: 250 - protein, 13 aa, Artificial Sequence
  CB301_H3L1_E6 Light Chain CDR1
CRGNNIGSKRVHW

SEQ ID NO: 251 - protein, 10 aa, Artificial Sequence
  CB301_H3L1_E6 Light Chain CDR2
SYNHRPSGVP

SEQ ID NO: 252 - protein, 14 aa, Artificial Sequence
  CB301_H3L1_E6 Light Chain CDR3
YCNTWDDSLEGPVF

SEQ ID NO: 253 - DNA, 31 bp, Artificial Sequence
  CB301_H3L1_F4 Heavy Chain CDR1
tcagcggctacgcaatgagctgggtcagaca

SEQ ID NO: 254 - DNA, 43 bp, Artificial Sequence; identical to SEQ ID NO: 110
  CB301_H3L1_F4 Heavy Chain CDR2

SEQ ID NO: 255 - DNA, 43 bp, Artificial Sequence
  CB301_H3L1_F4 Heavy Chain CDR3
actgcgcacgtagtcctagcggtctgttcgactactggggaca

SEQ ID NO: 256 - DNA, 37 bp, Artificial Sequence
  CB301_H3L1_F4 Light Chain CDR1
gctgcggtggtaacaacatcggtagcaagcgtgtgca

SEQ ID NO: 257 - DNA, 31 bp, Artificial Sequence
  CB301_H3L1_F4 Light Chain CDR2
acaacactagcaacaagcatagcggtgtgcc

SEQ ID NO: 258 - DNA, 37 bp, Artificial Sequence
  CB301_H3L1_F4 Light Chain CDR3
actgcagcagctacctacagcagcactctctgttcgg

SEQ ID NO: 259 - protein, 12 aa, Artificial Sequence
  CB301_H3L1_F4 Heavy Chain CDR1
FTFSGYAMSWVR

SEQ ID NO: 260 - protein, 13 aa, Artificial Sequence
  CB301_H3L1_F4 Heavy Chain CDR2
AISGSGGSTYYAD

SEQ ID NO: 261 - protein, 13 aa, Artificial Sequence
  CB301_H3L1_F4 Heavy Chain CDR3
YCARSPSGLFDYW

SEQ ID NO: 262 - protein, 13 aa, Artificial Sequence
  CB301_H3L1_F4 Light Chain CDR1
CGGNNIGSKRVHW

SEQ ID NO: 263 - protein, 10 aa, Artificial Sequence
  CB301_H3L1_F4 Light Chain CDR2
NTSNKHSGVP

SEQ ID NO: 264 - protein, 12 aa, Artificial Sequence
  CB301_H3L1_F4 Light Chain CDR3
YCSSYLQQHSLF

SEQ ID NO: 265 - DNA, 29 bp, Artificial Sequence
  CB301_H3L1_G11 Heavy Chain CDR1
agcagctacgcaatgagctgggtcagaca

SEQ ID NO: 266 - DNA, 43 bp, Artificial Sequence; identical to SEQ ID NO: 110
  CB301_H3L1_G11 Heavy Chain CDR2

SEQ ID NO: 267 - DNA, 49 bp, Artificial Sequence
  CB301_H3L1_G11 Heavy Chain CDR3
actgcacacgtttcgtgggtgcaatcggtgcattcgactactggggaca

SEQ ID NO: 268 - DNA, 37 bp, Artificial Sequence
  CB301_H3L1_G11 Light Chain CDR1
gctgcagtggtaacaacatcggtagccgtagcgtgca

SEQ ID NO: 269 - DNA, 31 bp, Artificial Sequence; identical to SEQ ID NO: 221
  CB301_H3L1_G11 Light Chain CDR2

SEQ ID NO: 270 - DNA, 43 bp, Artificial Sequence
  CB301_H3L1_G11 Light Chain CDR3
actgcgcagcatgggacgacagcctgagcggtcctgtgttcgg

SEQ ID NO: 271 - protein, 12 aa, Artificial Sequence
  CB301_H3L1_G11 Heavy Chain CDR1
FTFSSYAMSWVR

SEQ ID NO: 272 - protein, 13 aa, Artificial Sequence
  CB301_H3L1_G11 Heavy Chain CDR2
AISGSGGSTYYAD

SEQ ID NO: 273 - protein, 15 aa, Artificial Sequence
  CB301_H3L1_G11 Heavy Chain CDR3
YCTRFVGAIGAFDYW

SEQ ID NO: 274 - protein, 13 aa, Artificial Sequence
  CB301_H3L1_G11 Light Chain CDR1
CSGNNIGSRSVHW

SEQ ID NO: 275 - protein, 10 aa, Artificial Sequence
  CB301_H3L1_G11 Light Chain CDR2
RNNQRPSGVP

SEQ ID NO: 276 - protein, 14 aa, Artificial Sequence
  CB301_H3L1_G11 Light Chain CDR3
YCAAWDDSLSGPVF

SEQ ID NO: 277 - DNA, 31 bp, Artificial Sequence
  CB301_OPALTL_B5 Heavy Chain CDR1
tcagccattacgcaatgagctgggtcagaca

SEQ ID NO: 278 - DNA, 43 bp, Artificial Sequence; identical to SEQ ID NO: 110
  CB301_OPALTL_B5 Heavy Chain CDR2

SEQ ID NO: 279 - DNA, 55 bp, Artificial Sequence
  CB301_OPALTL_B5 Heavy Chain CDR3
actgcgcacgtggttgggacagccctactctgacatacttcgacagctggggaca

SEQ ID NO: 280 - DNA, 43 bp, Artificial Sequence
  CB301_OPALTL_B5 Light Chain CDR1
gctgcagcggtactagcagcaacatcggtaacaacgacgtgag

SEQ ID NO: 281 - DNA, 31 bp, Artificial Sequence
  CB301_OPALTL_B5 Light Chain CDR2
accaggacactaagcgtcctagcggtgtgcc

SEQ ID NO: 282 - DNA, 43 bp, Artificial Sequence; identical to SEQ ID NO: 270
  CB301_OPALTL_B5 Light Chain CDR3

SEQ ID NO: 283 - protein, 12 aa, Artificial Sequence
  CB301_OPALTL_B5 Heavy Chain CDR1
FTFSHYAMSWVR

SEQ ID NO: 284 - protein, 13 aa, Artificial Sequence
  CB301_OPALTL_B5 Heavy Chain CDR2
AISGSGGSTYYAD

SEQ ID NO: 285 - protein, 17 aa, Artificial Sequence
  CB301_OPALTL_B5 Heavy Chain CDR3
YCARGWDSPTLTYFDSW

SEQ ID NO: 286 - protein, 15 aa, Artificial Sequence
  CB301_OPALTL_B5 Light Chain CDR1
CSGTSSNIGNNDVSW

SEQ ID NO: 287 - protein, 10 aa, Artificial Sequence
  CB301_OPALTL_B5 Light Chain CDR2
QDTKRPSGVP

SEQ ID NO: 288 - protein, 14 aa, Artificial Sequence
  CB301_OPALTL_B5 Light Chain CDR3
YCAAWDDSLSGPVF

SEQ ID NO: 289 - DNA, 27 bp, Artificial Sequence
  CB301_OPALTL_E6 Heavy Chain CDR1
agcagctacggtatgcattgggtcaga

SEQ ID NO: 290 - DNA, 39 bp, Artificial Sequence
  CB301_OPALTL_E6 Heavy Chain CDR2
gcaatcagcggtagcggtggttacacttactacgcagac

SEQ ID NO: 291 - DNA, 36 bp, Artificial Sequence
  CB301_OPALTL_E6 Heavy Chain CDR3
tgcgcacgctggcattacagcttcgactactgggga

SEQ ID NO: 292 - DNA, 39 bp, Artificial Sequence
  CB301_OPALTL_E6 Light Chain CDR1
tgcagcggtagcagcagcaacatcggtaacaactacgtg

SEQ ID NO: 293 - DNA, 27 bp, Artificial Sequence
  CB301_OPALTL_E6 Light Chain CDR2
cgcaacaaccagcgccctagtggtgtg

SEQ ID NO: 294 - DNA, 33 bp, Artificial Sequence
  CB301_OPALTL_E6 Light Chain CDR3
tgccagagctacgacaacagcaacgtgctgttc

SEQ ID NO: 295 - protein, 12 aa, Artificial Sequence
  CB301_OPALTL_E6 Heavy Chain CDR1
FTFSSYGMHWVR

SEQ ID NO: 296 - protein, 13 aa, Artificial Sequence
  CB301_OPALTL_E6 Heavy Chain CDR2
AISGSGGYTYYAD

SEQ ID NO: 297 - protein, 12 aa, Artificial Sequence
  CB301_OPALTL_E6 Heavy Chain CDR3
YCARWHYSFDYW

SEQ ID NO: 298 - protein, 15 aa, Artificial Sequence
  CB301_OPALTL_E6 Light Chain CDR1
CSGSSSNIGNNYVSW

SEQ ID NO: 299 - protein, 10 aa, Artificial Sequence
  CB301_OPALTL_E6 Light Chain CDR2
RNNQRPSGVP

SEQ ID NO: 300 - protein, 12 aa, Artificial Sequence
  CB301_OPALTL_E6 Light Chain CDR3
YCQSYDNSNVLF

SEQ ID NO: 301 - DNA, 348 bp, Artificial Sequence
  CK1 Heavy chain variable region
gaagtgcagctgctggaaagtggaggtggactggtgcagcctggcggcagcctgcgcctgagctgtgccgccagcggattcaccttcagccgctatgccatgacctgggttcgccaagcacctggcaaaggcctggaatgggtgagcagcatgagcggcaccggcggcaccacctattatgccgatagcgtgaaaggtcgctttaccatcagccgcgataacagcaaaaacaccctgtatctgcagatgaacagcctgcgcgccgaggacaccgcagtctactactgtgcccgcggcgcctatggctttgatcattggggacaaggtactctggtgaccgtgagcagc

SEQ ID NO: 302 - DNA, 321 bp, Artificial Sequence
  CK1 Light Chain Variable Region
gaaatcgtgctgacccagagccctggcaccctgagcctgagccctggcgaacgcgcaacactgtcatgccgcgccagccagagcatcggcaactatctgaactggtatcagcagaaaccaggtcaggctccacgtctgctgatctatgatgccagcaacctggaaaccggcatccctgatcgcttctcaggatctggaagcggtaccgattttaccctgaccatcagccgcctggaacctgaggactttgccgtgtattattgtcagcagagtagcgccatcccttataccttcggtcagggcactaaagtggaaatcaaa

SEQ ID NO: 303 - protein, 116 aa, Artificial Sequence
  CK1 Heavy Chain Variable Region
EVQLLESGGGLVQPGGSLRLSCAASGFTFSRYAMTWVRQAPGKGLEWVSSMSGTGGTTYYADSVKGRFTISRDNSKNTLYLQMNSLRAEDTAVYYCARGAYGFDHWGQGTLVTVSS

SEQ ID NO: 304 - protein, 107 aa, Artificial Sequence
  CK1 Light Chain Variable Region
EIVLTQSPGTLSLSPGERATLSCRASQSIGNYLNWYQQKPGQAPRLLIYDASNLETGIPDRFSGSGSGTDFTLTISRLEPEDFAVYYCQQSSAIPYTFGQGTKVEIK

SEQ ID NO: 305 - DNA, 348 bp, Artificial Sequence
  CK2 Heavy Chain Variable Region
gaagtgcagctgctggaaagtggaggtggactggtgcagcctggcggcagcctgcgcctgagctgtgccgccagcggattcaccttcagcagctatggcatgcattgggttcgccaagcacctggcaaaggcctggaatgggtgagcgccatcagcggcagcggcaccagcatctattatgccgatagcgtgaaaggccgctttaccatcagccgcgataacagcaaaaacaccctgtatctgcagatgaacagcctgcgcgccgaggacaccgcagtctactactgtgcccgcggcggcaccgcctttgattattggggacaaggtactctggtgaccgtgagcagc

SEQ ID NO: 306 - DNA, 321 bp, Artificial Sequence
  CK2 Light Chain Variable Region
gaaatcgtgctgacccagagccctggcaccctgagcctgagccctggcgaacgcgcaacactgtcatgccgcgccagccagagatcagacaactatctggcctggtatcagcagaaaccaggtcaggctccacgtctgctgatctatgatgccagcaaccgcgccaccggcatccctgatcgcttctcaggatctggaagcggtaccgattttaccctgaccatcagccgcctggaacctgaggactttgccgtgtattattgtcagcagagctatagcaccccttttaccttcggtcagggcactaaagtggaaaccaaa

SEQ ID NO: 307 - protein, 116 aa, Artificial Sequence
  CK2 Heavy Chain Variable Region
EVQLLESGGGLVQPGGSLRLSCAASGFTFSSYGMHWVRQAPGKGLEWVSAISGSGTSIYYADSVKGRFTISRDNSKNTLYLQMNSLRAEDTAVYYCARGGTAFDYWGQGTLVTVSS

SEQ ID NO: 308 - protein, 107 aa, Artificial Sequence
  CK2 Light Chain Variable Region
EIVLTQSPGTLSLSPGERATLSCRASQRSDNYLAWYQQKPGQAPRLLIYDASNRATGIPDRFSGSGSGTDFTLTISRLEPEDFAVYYCQQSYSTPFTFGQGTKVETK

SEQ ID NO: 309 - DNA, 357 bp, Artificial Sequence
  CK3 Heavy Chain Variable Region
cgagtgcagctgctggaaagtggaggtggactggtgcagcctggcggcagcctgcgcctgagctgtgccgccagcggattcaccttcagcagctatgccatcagctgggttcgccaagcacctggcaaaggcctggaatgggtgagcgccaccagcggcagcggccgcgccacctattatgccgatagcgtgaaaggccgctttaccatcagccgcgataacagcaaaaacaccctgtatctgcagatgaacagcctgcgcgccgaggacaccgcagtctactactgtgcgcgcgatacctggtgggaaggctattttgatctgtggggacaaggtactctggtgaccgtgagcagc

SEQ ID NO: 310 - DNA, 318 bp, Artificial Sequence
  CK3 Light Chain Variable Region
gaaatcgtgctgacccagagccctggcaccctgagcctgagccctggcgaacgcgcaacactgtcatgccaggccagccatatcagcacccatctgaactggtatcagcagaaaccaggtcaggctccacgtctgctgatctatggcgccagcagccgcgccaccggcatccctgatcgcttctcaggatctggaagcggtaccgattttaccctgaccatcagccgcctggaacctgaggactttgccgtgtattattgtcagcagtataacacctatcctcctaccttcggtcagggcactaaagtggaaatcaaa

SEQ ID NO: 311 - protein, 119 aa, Artificial Sequence
  CK3 Heavy Chain Variable Region
RVQLLESGGGLVQPGGSLRLSCAASGFTFSSYAISWVRQAPGKGLEWVSATSGSGRATYYADSVKGRFTISRDNSKNTLYLQMNSLRAEDTAVYYCARDTWWEGYFDLWGQGTLVTVSS

SEQ ID NO: 312 - protein, 106 aa, Artificial Sequence
  CK3 Light Chain Variable Region
EIVLTQSPGTLSLSPGERATLSCQASHISTHLNWYQQKPGQAPRLLIYGASSRATGIPDRFSGSGSGTDFTLTISRLEPEDFAVYYCQQYNTYPPTFGQGTKVEIK

SEQ ID NO: 313 - DNA, 348 bp, Artificial Sequence
  CL4 Heavy Chain Variable Region
cgagtgcagctgctggaaagtggaggtggactggtgcagcctggcggcagcctgcgcctgagctgtgccgccagcggattcaccttcggcagcaactatatgagctgggttcgccaagcacctggcaaaggcctggaatgggtgagcaccatcagcggcagcggcaccagcacctattatgccgatagcttgaaaggccgctttaccatcagccgcgataacagcaaaaacaccctgtatctgcagatgaacagcctgcgcgccgaggacaccgcagtctactactgtgcccgcggcatgtggggcatggatgtgtggggacaaggtactctggtgaccgtgagcagc

SEQ ID NO: 314 - DNA, 312 bp, Artificial Sequence
  CL4 Light Chain Variable Region
cagagcgtgctgacccagcctcctagcgcctccggtacaccaggacagcgcgtgactattagctgtaccggcaaacatcggcacaccgtgaactggtaccagctactgcctggaactgcacctaagctgctgatctatctggatagcgaacgccctagcggcgtacctgatcgctttagcggtagcaaatcaggcaccagcgccagcctggccatcagcggccttcgctccgaagatgaagccgattattattgtcagagctatgatagcagcagcgtggtgtttggtggcggtaccaagctgaccgtgctg

SEQ ID NO: 315 - protein, 116 aa, Artificial Sequence
  CL4 Heavy Chain Variable Region
RVQLLESGGGLVQPGGSLRLSCAASGFTFGSNYMSWVRQAPGKGLEWVSTISGSGTSTYYADSLKGRFTISRDNSKNTLYLQMNSLRAEDTAVYYCARGMWGMDVWGQGTLVTVSS

SEQ ID NO: 316 - protein, 104 aa, Artificial Sequence
  CL4 Light Chain Variable Region
QSVLTQPPSASGTPGQRVTISCTGKHRHTVNWYQLLPGTAPKLLIYLDSERPSGVPDRFSGSKSGTSASLAISGLRSEDEADYYCQSYDSSSVVFGGGTKLTVL

SEQ ID NO: 317 - DNA, 351 bp, Artificial Sequence
  CL5 Heavy Chain Variable Region
cgagtgcagctgctggaaagtggaggtggactggtgcagcctggcggcagcctgcgcctgagctgtgccgccagcggattcaccttcagcagctatgccatgcattgggttcgccaagcacctggcaaaggcctggaatgggtgagcagcatcagcggcggcggctatggcacctattatgccgatagcgtgaaaggccgctttaccatcagccgcgataacagcaaaaacaccctgtatctgcagatgaacagcctgcgcgccgaggacaccgcagtctactactgtgcccgcagcaccgtgtgggcctttgatatctggggacaaggtactctggtgaccgtgagcagc

SEQ ID NO: 318 - DNA, 321 bp, Artificial Sequence
  CL5 Light Chain Variable Region
cagagcgtgctgacccagcctcctagcgcctccggtacaccaggacagcgcgtgactattagctgtagcggcaacaacatcggcagcaaaagcgtgcattggtaccagcaactgcctggaactgcacctaagctgctgatctatgatgtgagcaaacgccctagcgagcgtcctgatcgctttagcggtagcaaatcaggcaccagcgccagtctggccatcagcgaccttcgctccgaagatgaagccgattattattgtcagagctttgatagcagcggcacctggatctttggtggcggtaccaagctgaccgtgctg

SEQ ID NO: 319 - protein, 117 aa, Artificial Sequence
  CL5 Heavy Chain Variable Region
RVQLLESGGGLVQPGGSLRLSCAASGFTFSSYAMHWVRQAPGKGLEWVSSISGGGYGTYYADSVKGRFTISRDNSKNTLYLQMNSLRAEDTAVYYCARSTVWAFDIWGQGTLVTVSS

SEQ ID NO: 320 - protein, 107 aa, Artificial Sequence
  CL5 Light Chain Variable Region
QSVLTQPPSASGTPGQRVTISCSGNNIGSKSVHWYQQLPGTAPKLLIYDVSKRPSERPDRFSGSKSGTSASLAISDLRSEDEADYYCQSFDSSGTWIFGGGTKLTVL

SEQ ID NO: 321 - DNA, 357 bp, Artificial Sequence
  CL6 Heavy Chain Variable Region
gaggtgcagctgttggagtctggtggaggcttggtacagcctggaggttctcttcgcctctcctgtgcagcctccggattcactttcagcagctacggtatgcattgggtcagacaggcaccaggtaagggactggagtgggtctctgcaattagcggtagcggtggtagcacttactacgcagacagcgtgaagggtcgcttcaccatctcacgcgacaactccaagaacaccctgtacctgcagatgaacagccttcgcgcagaggacactgccgtgtattactgcgcagtcagtggtgcaggtcgtggtttcttcgactactggggacaaggtactctggtcactgtctcctca

SEQ ID NO: 322 - DNA, 327 bp, Artificial Sequence
  CL6 Light Chain Variable Region
cagtctgtgctgactcagccaccttcagcatctggtactccaggtcagcgcgtcaccatcagctgcagcggtagcagcagcaacattggtagcaactacgtgtactggtatcagcaactcccaggcaccgctcctaagctcctgatttacgaggacaacaagcgtcctagtggtgtgcctgatcgcttttctgggtccaagtctggcacctcagcctctctggctatcagtggacttcgctccgaggacgaggctgactattactgcagcagctacactagcagcagcactgtgatcttcggcggtgggaccaaactgaccgtccta

SEQ ID NO: 323 - protein, 119 aa, Artificial Sequence
  CL6 Heavy Chain Variable Region
EVQLLESGGGLVQPGGSLRLSCAASGFTFSSYGMHWVRQAPGKGLEWVSAISGSGGSTYYADSVKGRFTISRDNSKNTLYLQMNSLRAEDTAVYYCAVSGAGRGFFDYWGQGTLVTVSS

SEQ ID NO: 324 - protein, 109 aa, Artificial Sequence
  CL6 Light Chain Variable Region
QSVLTQPPSASGTPGQRVTISCSGSSSNIGSNYVYWYQQLPGTAPKLLIYEDNKRPSGVPDRFSGSKSGTSASLAISGLRSEDEADYYCSSYTSSSTVIFGGGTKLTVL

SEQ ID NO: 325 - DNA, 351 bp, Artificial Sequence
  CL7 Heavy Chain Variable Region
gaggtgcagctgttggagtctggtggaggcttggtacagcctggaggttctcttcgcctctcctgtgcagcctccggattcactttcagccgctacgcaatgagctgggtcagacaggcaccaggtaagggactggagtgggtctctgcaattagcggtagcggtggtagcacttactacgcagacagcgtgaagggtcgcttcaccatctcacgcgacaactccaagaacaccctgtacctgcagatgaacagccttcgcgcagaggacactgccgtgtattactgcgcacgtagcagccagggtatcttcgacatctggggacaaggtactctggtcactgtctcctca

SEQ ID NO: 326 - DNA, 324 bp, Artificial Sequence
  CL7 Light Chain Variable Region
cagtctgtgctgactcagccaccttcagcatctggtactccaggtcagcgcgtcaccatcagctgcagtggtaacaatatcggtactagacgcgtgcattggtatcagcaactcccagacaccgctcctaagctcctgatttacagtaagaacaaccgtcctagtggtgtgcctgatcgcttttctgggtccaagtctggcacctcagcctctctggctatcagtggacttcgctccgaggacgaggctgactattactgcgcagcatgggacgacagcctgagcggtcctgtgttcggcggtgggaccaaactgaccgtccta

SEQ ID NO: 327 - protein, 117 aa, Artificial Sequence
  CL7 Heavy Chain Variable Region
EVQLLESGGGLVQPGGSLRLSCAASGFTFSRYAMSWVRQAPGKGLEWVSAISGSGGSTYYADSVKGRFTISRDNSKNTLYLQMNSLRAEDTAVYYCARSSQGIFDIWGQGTLVTVSS

SEQ ID NO: 328 - protein, 108 aa, Artificial Sequence
  CL7 Light Chain Variable Region
QSVLTQPPSASGTPGQRVTISCSGNNIGTRRVHWYQQLPDTAPKLLIYSKNNRPSGVPDRFSGSKSGTSASLAISGLRSEDEADYYCAAWDDSLSGPVFGGGTKLTVL

SEQ ID NO: 329 - DNA, 354 bp, Artificial Sequence
  CL8 Heavy Chain Variable Region
gaggtgcagctgttggagtctggtggaggcttggtacagcctggaggttctcttcgcctctcctgtgcagcctccggattcactttcagcagctacgcaatgagctgggtcagacaggcaccaggtaagggactggagtgggtctctgcaattagcggtagcggtggtagcacttactacgcagacagcgtgaagggtcgcttcaccatctcacgcaacaactccaagaacaccctgtacctgcagatgaacagccttcgcgcagaggacactgccgtgtattactgcgcacgtagcggtcgttacgcagacttgacatctgggggacaaggtactctggtcactgtctcctca

SEQ ID NO: 330 - DNA, 327 bp, Artificial Sequence
  CL8 Light Chain Variable Region
cagtctgtgctgactcagccaccttcagcatctggtactccaggtcagcgcgtcaccatcagctgcagcggtagcaacagcaacatcggtaacaactacgtgagctggtatcagcaactcccagacacccctcctaagctcctgatttacgacaacaacaagcgtcctagtggtgtgcctgatcgcttttctgggtccaagtctggcacctcagcctctctggctatcagtggacttcgctccgaggacgaggctgactattactgcagcagctacactagcagcagcactgtgatgttcggcggtgggaccaaactgaccgtccta

SEQ ID NO: 331 - protein, 118 aa, Artificial Sequence
  CL8 Heavy Chain Variable Region
EVQLLESGGGLVQPGGSLRLSCAASGFTFSSYAMSWVRQAPGKGLEWVSAISGSGGSTYYADSVKGRFTISRNNSKNTLYLQMNSLRAEDTAVYYCARSGRYADLTSGGQGTLVTVSS

SEQ ID NO: 332 - protein, 109 aa, Artificial Sequence
  CL8 Light Chain Variable Region
QSVLTQPPSASGTPGQRVTISCSGSNSNIGNNYVSWYQQLPDTPPKLLIYDNNKRPSGVPDRFSGSKSGTSASLAISGLRSEDEADYYCSSYTSSSTVMFGGGTKLTVL

SEQ ID NO: 333 - DNA, 351 bp, Artificial Sequence
  CL9 Heavy Chain Variable Region
gaggtgcagctgttggagtctggtggaggcttggtacagcctggaggttctcttcgcctctcctgtgcagcctccggattcactttcagcagctactactggagctgggtcagacaggcaccaggtaagggactggagtgggtctctgcaattagcggtagcggtggtagcacttactacgcagacagcgtgaagggtcgcttcaccatctcacgcgacaactccaagaacaccctgtacctgcagatgaacagccttcgcgcagaggacactgccgtgtattactgcgcacgtatcgacgtgtacggtttcgacatctggggacaaggtactctggtcactgtctcctca

SEQ ID NO: 334 - DNA, 327 bp, Artificial Sequence
  CL9 Light Chain Variable Region
cagtctgtgctgactcagccaccttcagcatctggtactccaggtcagcgcgtcaccatcagctgcagcggtagcactagcaacatcggtactaactacgtgtactggtatcagcaactcccaggcaccgctcctaagctcctgatttacgacaacaacaaccgtcctagtggtgtgcctgatcgcttttctgggtccaagtctggcacctcagcctctctggctatcagtggacttcgctccgaggacgaggctgactattactgccagacttgggacagcagcactgacgtagtgttcggcggtgggaccaaactgaccgtccta

SEQ ID NO: 335 - protein, 117 aa, Artificial Sequence
  CL9 Heavy Chain Variable Region
EVQLLESGGGLVQPGGSLRLSCAASGFTFSSYYWSWVRQAPGKGLEWVSAISGSGGSTYYADSVKGRFTISRDNSKNTLYLQMNSLRAEDTAVYYCARIDVYGFDIWGQGTLVTVSS

SEQ ID NO: 336 - protein, 109 aa, Artificial Sequence
  CL9 Light Chain Variable Region
QSVLTQPPSASGTPGQRVTISCSGSTSNIGTNYVYWYQQLPGTAPKLLIYDNNNRPSGVPDRFSGSKSGTSASLAISGLRSEDEADYYCQTWDSSTDVVFGGGTKLTVL

SEQ ID NO: 337 - DNA, 348 bp, Artificial Sequence
  CL10 Heavy Chain Variable Region
gaggtgcagctgttggagtctggtggaggcttggtacagcctggaggttctcttcgcctctcctgtgcagcctccggattcactttcagcagctacggtatgcattgggtcagacaggcaccaggtaagggactggagtgggtctctgcaattagcggtagcggtggtagcacttactacgcagacagcgtgaagggtcgcttcaccatctcacgcgacaactccaagaacaccctgtacctgcagatgaacagccttcgcgcagaggacactgccgtgtattactgcgcaagcggttacggtctgatggacgtgtggggacaaggtactctggtcactgtctcctca

SEQ ID NO: 338 - DNA, 324 bp, Artificial Sequence
  CL10 Light Chain Variable Region
tctgtgctgactcagccaccttcagcatctggtactccaggtcagcgcgtcaccatcagctgcactcgtagcagcggtatcatcgcaagcaactacgtgcagtggtatcagcaactcccaggcaccgctcctaagctcctgatttaccgcaacaaccagcgccctagtggtgtgcctgatcgcttttctgggtccaagtctggcacctcagcctctctggctatcagtggacttcgctccgaggacgaggctgactattactgcagcagctacgcaggtaacaacaacctggtgttcggcggtgggaccaaactgaccgtccta

SEQ ID NO: 339 - protein, 116 aa, Artificial Sequence
  CL10 Heavy Chain Variable Region
EVQLLESGGGLVQPGGSLRLSCAASGFTFSSYGMHWVRQAPGKGLEWVSAISGSGGSTYYADSVKGRFTISRDNSKNTLYLQMNSLRAEDTAVYYCASGYGLMDVWGQGTLVTVSS

SEQ ID NO: 340 - protein, 109 aa, Artificial Sequence
  CL10 Light Chain Variable Region
QSVLTQPPSASGTPGQRVTISCTRSSGIIASNYVQWYQQLPGTAPKLLIYRNNQRPSGVPDRFSGSKSGTSASLAISGLRSEDEADYYCSSYAGNNNLVFGGGTKLTVL

SEQ ID NO: 341 - DNA, 348 bp, Artificial Sequence
  SK11 Heavy Chain Variable Region
cgagtgcagctgctggaaagtggaggtggactggtgcagcctggcggcagcctgcgcctgagctgtgccgccagcggattcaccttcagcacctatggcatgcattgggttcgccaagcacctggcaaaggcctggaatgggtgagcgccatcagcggcagcggcggcagcacctattatgccgatagcgtgaaaggccgctttaccatcagccgcgataacagcaaaaacaccctgtatctgcagatgaacagcctgcgcgccgaggacaccgcagtctactactgtgcccgcggcctgagcggccttgattattggggacaaggtactctggtgaccgtgagcagc

SEQ ID NO: 342 - DNA, 321 bp, Artificial Sequence
  SK11 Light Chain Variable Region
gaaatcgtgctgacccagagccctggcaccctgagcctgagccctggcgaacgcgcaacactgtcatgccgctccagccagggcatcaccaactatctggcctggtatcagcagaaaccaggtcaggctccacgtctgctgatctatgatgccagcaaccgcgccaccggcatccctgatcgcttctcaggatctggaagcggtaccgattttaccctgaccatcagccgcctggaacctgaggactttgccgtgtattattgtcagcagagctatagcacccctctgaccttcggtcagggcactaaagtggaaatcaaa

SEQ ID NO: 343 - protein, 116 aa, Artificial Sequence
  SK11 Heavy Chain Variable Region
RVQLLESGGGLVQPGGSLRLSCAASGFTFSTYGMHWVRQAPGKGLEWVSAISGSGGSTYYADSVKGRFTISRDNSKNTLYLQMNSLRAEDTAVYYCARGLSGLDYWGQGTLVTVSS

SEQ ID NO: 344 - protein, 107 aa, Artificial Sequence
  SK11 Light Chain Variable Region
EIVLTQSPGTLSLSPGERATLSCRSSQGITNYLAWYQQKPGQAPRLLIYDASNRATGIPDRFSGSGSGTDFTLTISRLEPEDFAVYYCQQSYSTPLTFGQGTKVEIK

SEQ ID NO: 345 - DNA, 348 bp, Artificial Sequence
  SK12 Heavy Chain Variable Region
cgagtgcagctgctggaaagtggaggtggactggtgcagcctggcggcagcctgcgcctgagctgtgccgccagcggattcaccttcagcagctatgccatgcattgggttcgccaagcacctggcaaaggcctggaatgggtgagcgccatcagcggcagcggcggcgatacctatcatgccgatagcgtgaaaggccgctttaccatcagccgcgataacagcaaaaacaccctgtatctgcagatgaacagcctgcgcgccgaggacaccgcagtctactactgtacccgcggcctgagcggctttgattattggggacaaggtactctggtgaccgtgagcagc

SEQ ID NO: 346 - DNA, 321 bp, Artificial Sequence
  SK12 Light Chain Variable Region
gaaatcgtgctgacccagagccctggcaccctgagcctgagccctggcgaacgcgcaacactgtcatgccgcgccagccagagcatcagcagctatctgaactggtatcagcagaaaccaggtcaggctccacgtctgctgatctatgatgccagcaaccgcgcccctggcatccctgatcgcttctcaggatctggaagcggtaccgattttaccctgaccatcagccgcctggaacctgaggactttgccgtgtattattgtcagcagagctatagcatccctatcaccttcggtcagggcactaaagtggaaatcaaa

SEQ ID NO: 347 - protein, 116 aa, Artificial Sequence
  SK12 Heavy Chain Variable Region
RVQLLESGGGLVQPGGSLRLSCAASGFTFSSYAMHWVRQAPGKGLEWVSAISGSGGDTYHADSVKGRFTISRDNSKNTLYLQMNSLRAEDTAVYYCTRGLSGFDYWGQGTLVTVSS

SEQ ID NO: 348 - protein, 110 aa, Artificial Sequence
  SK12 Light Chain Variable Region
EIVLTQSPGTLSLSPGERATLSCRASQSISSYLNWYQQKPGQAPRLLIYDASNRAPGIPDRFSGSGSGTDFTLTISRLEPEDFAVYYCQQSYSIPITFGQGTKVEIKFSD

SEQ ID NO: 349 - DNA, 348 bp, Artificial Sequence
  SK13 Heavy Chain Variable Region
cgagtgcagctgctggaaagtggaggtggactggtgcagcctggcggcagcctgcgcctgagctgtgccgccagcggattcaccttcagcgattatgccatgagctgggttcgccaagcacctggcaaaggcctggaatgggtgagcagcatcagcagcagcagcagctatatctactataccgatagcgtgaaaggccgctttaccatcagccgcgataacagcaaaaacaccctgtatctgcagatgaacagcctgcgcgccgaggacaccgcagtctactactgtgcccgcggcggctatggctttgattattggggacaaggtaccctggtgaccgtgagcagc

SEQ ID NO: 350 - DNA, 321 bp, Artificial Sequence
  SK13 Light Chain Variable Region
gaaatcgtgctgacccagagccctggcaccctgagcctgagccctggcgaacgcgcaacactgtcatgccgcgccagccagagcatcagcagctatctgaactggtatcagcagaaaccaggtcaggctccacgtctgctgatctatagcgccagcagccgcccacagggcatccccgatcgcttctcaggatctggaagcggtaccgattttaccctgaccatcagccgcctggaacctgaggactttgccgtgtattattgtcagcagtatgatgatctgccttttaccttcggtcagggcactaaagtggaaatcaaa

SEQ ID NO: 351 - protein, 116 aa, Artificial Sequence
  SK13 Heavy Chain Variable Region
RVQLLESGGGLVQPGGSLRLSCAASGFTFSDYAMSWVRQAPGKGLEWVSSISSSSSYIYYTDSVKGRFTISRDNSKNTLYLQMNSLRAEDTAVYYCARGGYGFDYWGQGTLVTVSS

SEQ ID NO: 352 - protein, 107 aa, Artificial Sequence
  SK13 Light Chain Variable Region
EIVLTQSPGTLSLSPGERATLSCRASQSISSYLNWYQQKPGQAPRLLIYSASSRPQGIPDRFSGSGSGTDFTLTISRLEPEDFAVYYCQQYDDLPFTFGQGTKVEIK

SEQ ID NO: 353 - DNA, 346 bp, Artificial Sequence
  SK14 Heavy Chain Variable Region
gaagtgcagctgctggaaagtggaggtggactggtgcagcctggcggcagcctgcgcctgagctgtgccgccagcggattcaccttcagcaactttgcgatcgcctgggttcgccaagcacctggcaaaggcctggaatgggtgagcgccatcagcggccgcggcaccagcacctattatgccgatagcgtgaaaggccgctttaccatcagccgcgataacagcaaaaacaccctgtatctgcagatgaacagcctgcgcgccgaggacaccgcagtctactactgtgcccgcggcgtgagcggctttgatagctggggacaaggtactctggtgaccgtgagca

SEQ ID NO: 354 - DNA, 321 bp, Artificial Sequence
  SK14 Light Chain Variable Region
gaaatcgtgctgacccagagccctggcaccctgagcctgagccctggcgaacgcgcaacactgtcatgccgcgccagccagagcatcagcagccatctggcctggtatcagcagaaaccaggtcaggctccacgtctgctgatctatgataccagcaaccgcgccaccggcatccctgatcgcttctcaggatctgggagcggtaccgattttaccctgaccatcagccgcctggaacctgaggactttgccgtgtactattgtcagcagagctatagcaccccttttaccttcggtcagggcactaaagtggaaatcaaa

SEQ ID NO: 355 - protein, 116 aa, Artificial Sequence
  SK14 Heavy Chain Variable Region
EVQLLESGGGLVQPGGSLRLSCAASGFTFSNFAIAWVRQAPGKGLEWVSAISGRGTSTYYADSVKGRFTISRDNSKNTLYLQMNSLRAEDTAVYYCARGVSGFDSWGQGTLVTVSS

SEQ ID NO: 356 - protein, 107 aa, Artificial Sequence
  SK14 Light Chain Variable Region
EIVLTQSPGTLSLSPGERATLSCRASQSISSHLAWYQQKPGQAPRLLIYDTSNRATGIPDRFSGSGSGTDFTLTISRLEPEDFAVYYCQQSYSTPFTFGQGTKVEIK

SEQ ID NO: 357 - DNA, 349 bp, Artificial Sequence
  SK15 Heavy Chain Variable Region
cgagtgcagctgctggaaagtggaggtggactggtgcagcctggcggcagcctgcgcctgagctgtgccgccagcggattcaccttcagcagctatgccatgcattgggttcgccaagcacctggcaaaggcctggaatgggtgagcgccatcaacggcagcggcggcagcacctattatgccgatagcgtgaaaggccgctttaccatcagccgcgataacagcaaaaacaccctgtatctgcagacgaacagcctgcgcgccgaggacaccgcagtctactactgtgcccgcggcctgcagggctttgattattggggacaaggtactctggtgaccgtgagcagca

SEQ ID NO: 358 - DNA, 321 bp, Artificial Sequence
  SK15 Light Chain Variable Region
gaaatcgtgctgacccagagccctggcaccctgagcctgagccctggcgaacgcgcaacactgtcatgccaggccagccaggatatcaccaactatctgaactggtatcagcagaaaccaggtcaggctccacgtctgctgatctatgatgccagcagcctggaaaccggcatccctgatcgtttctcaggatctggaagcggtaccgattttaccctgaccatcagccgcctggaacctgaggactttgccgtgtattattgtcagcagagctatagcacccctatcaccttcggtcagggcactaaagtggaaatcaaa

SEQ ID NO: 359 - protein, 116 aa, Artificial Sequence
  SK15 Heavy Chain Variable Region
RVQLLESGGGLVQPGGSLRLSCAASGFTFSSYAMHWVRQAPGKGLEWVSAINGSGGSTYYADSVKGRFTISRDNSKNTLYLQTNSLRAEDTAVYYCARGLQGFDYWGQGTLVTVSS

SEQ ID NO: 360 - protein, 107 aa, Artificial Sequence
  SK15 Light Chain Variable Region
EIVLTQSPGTLSLSPGERATLSCQASQDITNYLNWYQQKPGQAPRLLIYDASSLETGIPDRFSGSGSGTDFTLTISRLEPEDFAVYYCQQSYSTPITFGQGTKVEIK

SEQ ID NO: 361 - DNA, 349 bp, Artificial Sequence
  SK16 Heavy Chain Variable Region
cgagtgcagctgctggaaagtggaggtggactggtgcagcctggcggcagcctgcgcctgagctgtgccgccagcggattcaccttcagcagctatgccatgagctgggttcgccaagcacctggcaaaggcctggaatgggtgagcgccatcaacggcagcggcggcagcaccctgtatgccgatagcgtgaaaggccgctttaccatcagccgcgataacagcaaaaacaccctgtatctgcagatgaacagcctgcgcgccgaggacaccgcagtctactactgtgcccgcggcgtgagcggctttgatagctggggacaaggtactctggtgaccgtgagcagcg

SEQ ID NO: 362 - DNA, 321 bp, Artificial Sequence
  SK16 Light Chain Variable Region
gaaatcgtgctgacccagagccctggcaccctgagcctgagccctggcgaacgcgcaacactgtcatgccgcatcagccagagcatcagcagctatctgaactggtatcagcagaaaccaggtcaggctccacgtctgctgatctatgatgccagcctgcgcgccaccggcatccctgatcgcttctcaggatctggaagcggtaccgattttaccctgaccatcagccgcctggaacctgaggactttgccgtgtattattgtcagcagagctataaaacccctatcaccttcggtcagggcactaaagtggaaatcaaa

SEQ ID NO: 363 - protein, 116 aa, Artificial Sequence
  SK16 Heavy Chain Variable Region
RVQLLESGGGLVQPGGSLRLSCAASGFTFSSYAMSWVRQAPGKGLEWVSAINGSGGSTLYADSVKGRFTISRDNSKNTLYLQMNSLRAEDTAVYYCARGVSGFDSWGQGTLVTVSS

SEQ ID NO: 364 - protein, 107 aa, Artificial Sequence
  SK16 Light Chain Variable Region
EIVLTQSPGTLSLSPGERATLSCRISQSISSYLNWYQQKPGQAPRLLIYDASLRATGIPDRFSGSGSGTDFTLTISRLEPEDFAVYYCQQSYKTPITFGQGTKVEIK

SEQ ID NO: 365 - DNA, 349 bp, Artificial Sequence
  SK17 Heavy Chain Variable Region
gaagtgcagctgctggaaagtggaggtggactggtgcagcctggcggcagcctgcgcctgagctgtgccgccagcggattcaccttcagcagctattattggagctgggttcgccaagcacctggcaaaggcctggaatgggtgagcaccatcaccggcagcggcggcagcaccgattatgccaacagcgtgaaaggccgctttaccatcagccgcgataacagcaaaaacaccctgtatctgcagatgaacagcctgcgcgccgaggacaccgcagtctactactgtgccaccggcggcggcatctttgactattggggacaaggtactctggtgaccgtgagcagcg

SEQ ID NO: 366 - DNA, 321 bp, Artificial Sequence
  SK17 Light Chain Variable Region
gaaatcgtgctgacccagagccctggcaccctgagcctgagccctggcgaacgcgcaacactgtcatgccaggccagccagaccatcagcaactatctgaactggtatcagcagaaaccaggtcaggctccacgtctgctgatctatgatgccagcaaccgcgccaccggcatccctgatcgcttctcaggatctggaagcggtaccgattttaccctgaccatcagccgcctggaacctgaggactttgccgtgtattattgtcagcagtacaacagctatcctcctagcttcggtcagggcactaaagtggaaatcaaa

SEQ ID NO: 367 - protein, 116 aa, Artificial Sequence
  SK17 Heavy Chain Variable Region
EVQLLESGGGLVQPGGSLRLSCAASGFTFSSYYWSWVRQAPGKGLEWVSTITGSGGSTDYANSVKGRFTISRDNSKNTLYLQMNSLRAEDTAVYYCATGGGIFDYWGQGTLVTVSS

SEQ ID NO: 368 - protein, 107 aa, Artificial Sequence
  SK17 Light Chain Variable Region
EIVLTQSPGTLSLSPGERATLSCQASQTISNYLNWYQQKPGQAPRLLIYDASNRATGIPDRFSGSGSGTDFTLTISRLEPEDFAVYYCQQYNSYPPSFGQGTKVEIK

SEQ ID NO: 369 - DNA, 352 bp, Artificial Sequence
  SL18 Heavy Chain Variable Region
cgagtgcagctgctggaaagtggaggtggactggtgcagcctggcggcagcctgcgcctgagctgtgccgccagcggattcaccttcagcgattatcatatgcattgggttcgccaagcacctggcaaaggcctggaatgggtgagcaccatcagcagcagcggcggctatacctattatgccgaaagcgtgaaaagccgctttaccatcagccgcgataacagcaaaaacaccctgtatctgcagatgaacagcctgcgcgccgaggacaccgcagtctactactgtgcccgatcgatacgcctgcctctggattattggggacaaggtactctggtgaccgtgagcagca

SEQ ID NO: 370 - DNA, 321 bp, Artificial Sequence
  SL18 Light Chain Variable Region
cagagcgtgctgacccagcctcctagcgcctccggtacaccaggacagcgcgtgactattagctgtagcggcaacaacatcggcagcaaaggcgtgcattggtatcagcaactgcctggaactgcacctaagctgctgatctatgaagatagcaaacgccctagcggcgtgcgtgatcgctttagcggtagcaaatcaggcaccagcgccagcctggccatcagcggccttcgctccgaagatgaagccgattattattgtcagagctatgatagcaccaaaggcgtggtgtttggtggcggtaccaagctgaccgtgctg

SEQ ID NO: 371 - protein, 117 aa, Artificial Sequence
  SL18 Heavy Chain Variable Region
RVQLLESGGGLVQPGGSLRLSCAASGFTFSDYHMHWVRQAPGKGLEWVSTISSSGGYTYYAESVKSRFTISRDNSKNTLYLQMNSLRAEDTAVYYCARSIRLPLDYWGQGTLVTVSS

SEQ ID NO: 372 - protein, 107 aa, Artificial Sequence
  SL18 Light Chain Variable Region
QSVLTQPPSASGTPGQRVTISCSGNNIGSKGVHWYQQLPGTAPKLLIYEDSKRPSGVRDRFSGSKSGTSASLAISGLRSEDEADYYCQSYDSTKGVVFGGGTKLTVL

SEQ ID NO: 373 - DNA, 348 bp, Artificial Sequence
  CB301_H3L1_A10 Heavy Chain Variable Region
gaggtgcagctgttggagtctggtggaggcttggtacagtctggaggttctcttcgcctctcctgtgcagcctccggattcactttcagcagctacggtatgcattgggtcagacaggcaccaggtaagggactggagtgggtctctgcaattagcggtagcggtggtagcacttactacgcagacagcgtgaagggtcgcttcaccatctcacgcgacaactccaagaacaccctgtacctgcagatgaacagccttcgcgcagaggacactgccgtgtattactgcgtgcgtggttacggtgcaatggacgtgtggggacaaggtactctggtcactgtctcctca

SEQ ID NO: 374 - DNA, 327 bp, Artificial Sequence
  CB301_H3L1_A10 Light Chain Variable Region
cagtctgtgctgactcagccaccttcagcatctggtactccaggtcagcgcgtcaccatcagctgcactcgtagcagcggtagcatcgcaagcaactacgtgcagtggtatcagcaactcccaggcaccgctcctaagctcctgatttaccgcaacaaccagcgccctagtggtgtgcctgatcgcttttctgggtccaagtctggcacctcagcctctctggctatcagtggacttcgctccgaggacgaggctgactattactgcagcagctacactactagcagcactctggtgttcggcggtgggaccaaactgaccgtccta

SEQ ID NO: 375 - protein, 116 aa, Artificial Sequence
  CB301_H3L1_A10 Heavy Chain Variable Region
EVQLLESGGGLVQSGGSLRLSCAASGFTFSSYGMHWVRQAPGKGLEWVSAISGSGGSTYYADSVKGRFTISRDNSKNTLYLQMNSLRAEDTAVYYCVRGYGAMDVWGQGTLVTVSS

SEQ ID NO: 376 - protein, 109 aa, Artificial Sequence
  CB301_H3L1_A10 Light Chain Variable Region
QSVLTQPPSASGTPGQRVTISCTRSSGSIASNYVQWYQQLPGTAPKLLIYRNNQRPSGVPDRFSGSKSGTSASLAISGLRSEDEADYYCSSYTTSSTLVFGGGTKLTVL

SEQ ID NO: 377 - DNA, 348 bp, Artificial Sequence
  CB301_H3L1_A12 Heavy Chain Variable Region
gaggtgcagctgttggagtctggtggaggcttggtacagcctggaggttctcttcgcctctcctgtgcagcctccggattcactttcagcagctacgcaatgcattgggtcagacaggcaccaggtaagggactggagtgggtctctgcaattagcggtagcggtggtagcacttactacgcagacagcgtgaagggtcgcttcaccatctcacgcgacaactccaagaacaccctgtacctgcagatgaacagccttcgcgcaaaggacactgccgtgtattactgcgcaagcggctacggtctgatggacgtatggggacaaggtactctggtcactgtctcctca

SEQ ID NO: 378 - DNA, 330 bp, Artificial Sequence
  CB301_H3L1_A12 Light Chain Variable Region
cagtctgtgctgactcagccaccttcagcatctggtactccaggtcagcgcgtcaccatcagctgcactggtactagcagcgacgtgggtaactacaacctggtgagctggtatcagcaactcccaggcaccgctcctaagctcctgatttacagcaacaaccagcgccctagtggtgtgcctgatcgcttttctgggtccaagtctggcacctcagcctctctggctatcagtggacttcgctccgaggacgaggctgactattactgcagcagctacactggtagcaacgctctgttgttcggcggtgggaccaaactgaccgtccta

SEQ ID NO: 379 - protein, 116 aa, Artificial Sequence
  CB301_H3L1_A12 Heavy Chain Variable Region
EVQLLESGGGLVQPGGSLRLSCAASGFTFSSYAMHWVRQAPGKGLEWVSAISGSGGSTYYADSVKGRFTISRDNSKNTLYLQMNSLRAKDTAVYYCASGYGLMDVWGQGTLVTVSS

SEQ ID NO: 380 - protein, 110 aa, Artificial Sequence
  CB301_H3L1_A12 Light Chain Variable Region
QSVLTQPPSASGTPGQRVTISCTGTSSDVGNYNLVSWYQQLPGTAPKLLIYSNNQRPSGVPDRFSGSKSGTSASLAISGLRSEDEADYYCSSYTGSNALLFGGGTKLTVL

SEQ ID NO: 381 - DNA, 348 bp, Artificial Sequence
  CB301_H3L1_E6 Heavy Chain Variable Region
gaggtgcagctgttggagtctggtggaggcttggtacagcctggaggttctcttcgcctctcctgtgcagcctccggattcactttcagcagctacgcaatgagctgggtcagacaggcaccaggtaagggactggagtgggtctctgcaattagcggtagcggtggtagcacttactacgcagacagcgtgaagggtcgcttcaccatctcacgcgacaactccaagaacaccctgtacctgcagatgaacagccttcgcgcagaggacactgccgtgtattactgcgcacgctggcattacagcttcgactactggggacaaggtactctggtcactgtctcctca

SEQ ID NO: 382 - DNA, 324 bp, Artificial Sequence
  CB301_H3L1_E6 Light Chain Variable Region
cagtctgtgctgactcagccaccttcagcatctggtactccaggtcagcgcgtcaccatcagctgccgtggtaacaacatcggtagcaagcgtgtgcattggtatcagcaactcccaggcaccgctcctaagctcctgatttacagctacaaccaccgtcctagcggtgtgcctgatcgcttttctgggtccaagtctggcacctcagcctctctggctatcactggacttcgctccgaggacgaagctgactattactgcaacacttgggacgacagcctggagggtcctgtgttcggcggtgggaccaaactgaccgtccta

SEQ ID NO: 383 - protein, 116 aa, Artificial Sequence
  CB301_H3L1_E6 Heavy Chain Variable Region
EVQLLESGGGLVQPGGSLRLSCAASGFTFSSYAMSWVRQAPGKGLEWVSAISGSGGSTYYADSVKGRFTISRDNSKNTLYLQMNSLRAEDTAVYYCARWHYSFDYWGQGTLVTVSS

SEQ ID NO: 384 - protein, 108 aa, Artificial Sequence
  CB301_H3L1_E6 Light Chain Variable Region
QSVLTQPPSASGTPGQRVTISCRGNNIGSKRVHWYQQLPGTAPKLLIYSYNHRPSGVPDRFSGSKSGTSASLAITGLRSEDEADYYCNTWDDSLEGPVFGGGTKLTVL

SEQ ID NO: 385 - DNA, 352 bp, Artificial Sequence
  CB301_H3L1_F4 Heavy Chain Variable Region
gaggtgcagctgttggagtctggtggaggcttggtacagcctggaggttctcttcgcctctcctgtgcagcctccggattcactttcagcggctacgcaatgagctgggtcagacaggcaccaggtaagggactggagtgggtctctgcaattagcggtagcggtggtagcacttactacgcagacagcgtgaagggtcgcttcaccatctcacgcgacaactccaagaacaccctgtacctgcagatgaacagccttcgcgcagaggacactgccgtgtattactgcgcacgtagtcctagcggtctgttcgactactggggacaaggtactctggtcactgtctcctcag

SEQ ID NO: 386 - DNA, 318 bp, Artificial Sequence
  CB301_H3L1_F4 Light Chain Variable Region
cagtctgtgctgactcagccaccttcagcatctggtactccaggtcagcgcgtcaccatcagctgcggtggtaacaacatcggtagcaagcgtgtgcattggtatcagcaactcccaggcaccgctcctaagctcctgatttacaacactagcaacaagcatagcggtgtgcctgatcgcttttctgggtccaagtctggcacctcagcctctctggctatcagtggacttcgctccgaggacgaggctgactattactgcagcagctacctacagcagcactctctgttcggcggtgggaccaaactaaccgtccta

SEQ ID NO: 387 - protein, 117 aa, Artificial Sequence
  CB301_H3L1_F4 Heavy Chain Variable Region
EVQLLESGGGLVQPGGSLRLSCAASGFTFSGYAMSWVRQAPGKGLEWVSAISGSGGSTYYADSVKGRFTISRDNSKNTLYLQMNSLRAEDTAVYYCARSPSGLFDYWGQGTLVTVSS

SEQ ID NO: 388 - protein, 106 aa, Artificial Sequence
  CB301_H3L1_F4 Light Chain Variable Region
QSVLTQPPSASGTPGQRVTISCGGNNIGSKRVHWYQQLPGTAPKLLIYNTSNKHSGVPDRFSGSKSGTSASLAISGLRSEDEADYYCSSYLQQHSLFGGGTKLTVL

SEQ ID NO: 389 - DNA, 360 bp, Artificial Sequence
  CB301_H3L1_G11 Heavy Chain Variable Region
gaggtgcagctgttggagtctggtggaggcttggtacagcctggaggttcctcttccgcctcctcctgtgcagcctccggattcactttcagcagctacgcaatgagctgggtcagacaggcaccaggtaagggactggagtgggtctctgcaattagcggtagcggtggtagcacttactacgcagacagcgtgaagggtcgcttcaccatctcacgcgacaactccaagaacaccctgtacctgcagatgaacagccttcgcgcagaggacactgccgtgtattactgcacacgtttcgtgggtgcaatcggtgcattcgactactggggacaaggtactctggtcactgtctcctca

SEQ ID NO: 390 - DNA, 324 bp, Artificial Sequence
  CB301_H3L1_G11 Light Chain Variable Region
cagtctgtgctgactcagccaccttcagcatctggtactccaggtcagcgcgtcaccatcagctgcagtggtaacaacatcggtagccgtagcgtgcattggtatcagcaactcccaggcaccgctcctaagctcctgatttaccgcaacaaccagcgccctagtggtgtgcctgatcgcttttctgggtccaagtctggcacctcagcctctctggctatcagtggacttcgctccgaggacgaggctgactattactgcgcagcatgggacgacagcctgagcggtcctgtgttcggcggtgggaccaaactgaccgtccta

SEQ ID NO: 391 - protein, 120 aa, Artificial Sequence
  CB301_H3L1_G11 Heavy Chain Variable Region
EVQLLESGGGLVQPGGSSSASSCAASGFTFSSYAMSWVRQAPGKGLEWVSAISGSGGSTYYADSVKGRFTISRDNSKNTLYLQMNSLRAEDTAVYYCTRFVGAIGAFDYWGQGTLVTVSS

SEQ ID NO: 392 - protein, 108 aa, Artificial Sequence
  CB301_H3L1_G11 Light Chain Variable Region
QSVLTQPPSASGTPGQRVTISCSGNNIGSRSVHWYQQLPGTAPKLLIYRNNQRPSGVPDRFSGSKSGTSASLAISGLRSEDEADYYCAAWDDSLSGPVFGGGTKLTVL

SEQ ID NO: 393 - DNA, 363 bp, Artificial Sequence
  CB301_OPALTL_B5 Heavy Chain Variable Region
gaggtgcagctgttggagtctggtggaggcttggtacagcctggaggttctcttcgcctctcctgtgcagcctccggattcactttcagccattacgcaatgagctgggtcagacaggcaccaggtaagggactggagtgggtctctgcaattagcggtagcggtggtagcacttactacgcagacagcgtgaagggtcgcttcaccatctcacgcgacaactccaagaacaccctgtacctgcagatgaacagccttcgcgcagaggacactgccgtgtattactgcgcacgtggttgggacagccctactctgacatacttcgacagctggggacaaggtactctggtcactgtctcctca

SEQ ID NO: 394 - DNA, 330 bp, Artificial Sequence
  CB301_OPALTL_B5 Light Chain Variable Region
cagtctgtgctgactcagccaccttcagcatctggtactccaggtcagcgcgtcaccatcagctgcagcggtactagcagcaacatcggtaacaacgacgtgagctggtatcagcaactcccaggcaccgctcctaagctcctgatttaccaggacactaagcgtcctagcggtgtgcctgatcgcttttctgggtccaagtctggcacctcagcctctctggctatcagtggacttcgctccgaggacgaggctgactattactgcgcagcatgggacgacagcctgagcggtcctgtgttcggcggtgggaccaaactgaccgtccta

SEQ ID NO: 395 - protein, 121 aa, Artificial Sequence
  CB301_OPALTL_B5 Heavy Chain Variable Region
EVQLLESGGGLVQPGGSLRLSCAASGFTFSHYAMSWVRQAPGKGLEWVSAISGSGGSTYYADSVKGRFTISRDNSKNTLYLQMNSLRAEDTAVYYCARGWDSPTLTYFDSWGQGTLVTVSS

SEQ ID NO: 396 - protein, 110 aa, Artificial Sequence
  CB301_OPALTL_B5 Light Chain Variable Region
QSVLTQPPSASGTPGQRVTISCSGTSSNIGNNDVSWYQQLPGTAPKLLIYQDTKRPSGVPDRFSGSKSGTSASLAISGLRSEDEADYYCAAWDDSLSGPVFGGGTKLTVL

SEQ ID NO: 397 - DNA, 348 bp, Artificial Sequence
  CB301_OPALTL_E6 Heavy Chain Variable Region
gaggtgcagctgttggagtctggtggaggcttggtacagcctggaggttctcttcgcctctcctgtgcagcctccggattcactttcagcagctacggtatgcattgggtcagacaggcaccaggtaagggactggagtgggtctctgcaatcagcggtagcggtggttacacttactacgcagacagcgtgaagggtcgcttcaccatctcacgcgacaactccaagaacaccctgtacctgcagatgaacagccttcgcgcagaggacactgccgtgtattactgcgcacgctggcattacagcttcgactactggggacaaggtactctggtcactgtctcctca

SEQ ID NO: 398 - DNA, 324 bp, Artificial Sequence
  CB301_OPALTL_E6 Light Chain Variable Region
cagtctgtgctgactcagccaccttcagcatctggtactccaggtcagcgcgtcaccatcagctgcagcggtagcagcagcaacatcggtaacaactacgtgagctggtatcagcaactcccaggcaccgctcctaagctcctgatttaccgcaacaaccagcgccctagtggtgtgcctgatcgcttttctgggtccaagtctggcacctcagcctctctggctatcagtggacttcgctccgaggacgaggctgactattactgccagagctacgacaacagcaacgtgctgttcggcggtgggaccaaactgaccgtccta

SEQ ID NO: 399 - protein, 116 aa, Artificial Sequence
  CB301_OPALTL_E6 Heavy Chain Variable Region
EVQLLESGGGLVQPGGSLRLSCAASGFTFSSYGMHWVRQAPGKGLEWVSAISGSGGYTYYADSVKGRFTISRDNSKNTLYLQMNSLRAEDTAVYYCARWHYSFDYWGQGTLVTVSS

SEQ ID NO: 400 - protein, 108 aa, Artificial Sequence
  CB301_OPALTL_E6 Light Chain Variable Region
QSVLTQPPSASGTPGQRVTISCSGSSSNIGNNYVSWYQQLPGTAPKLLIYRNNQRPSGVPDRFSGSKSGTSASLAISGLRSEDEADYYCQSYDNSNVLFGGGTKLTVL

SEQ ID NO: 401 - DNA, 489 bp, Artificial Sequence
  CD300c ECD
ggctattttcctctgagccaccccatgaccgtggcgggccccgtggggggatccctgagtgtgcagtgtcgctatgagaaggaacacaggaccctcaacaaattctggtgcagaccaccacagattctccgatgtgacaagattgtggagaccaaagggtcagcagggaaaaggaatggccgagtgtccatcagggacagtcctgcaaacctcagcttcacagtgaccctggagaatctcacagaggaggacgcaggcacctactggtgtggggtggatacaccgtggctccgagactttcatgatcccattgtcgaggttgaggtgtccgtgttcccggccgggacgaccacagcctccagcccccagagctccatgggcacctcaggtcctcccacgaagctgcccgtgcacacctggcccagcgtgaccagaaaggacagccccgaacccagcccacaccctggctccctgttcagcaatgtccgc

SEQ ID NO: 402 - protein, 163 aa, Artificial Sequence
  CD300c ECD
GYFPLSHPMTVAGPVGGSLSVQCRYEKEHRTLNKFWCRPPQILRCDKIVETKGSAGKRNGRVSIRDSPANLSFTVTLENLTEEDAGTYWCGVDTPWLRDFHDPIVEVEVSVFPAGTTTASSPQSSMGTSGPPTKLPVHTWPSVTRKDSPEPSPHPGSLFSNVR

SEQ ID NO: 403 - protein, 12 aa, Artificial Sequence
  Heavy chain CDR1 of anti-CD300c monoclonal antibody or antigen binding fragment thereof
  MISC_FEATURE (4): Xaa = G or S
  MISC_FEATURE (5): Xaa = S, R, or D
  MISC_FEATURE (6): Xaa = N or Y
  MISC_FEATURE (7): Xaa = Y, A, G, or H
  MISC_FEATURE (9): Xaa = S, or H
FTFXXXXMXWVR

SEQ ID NO: 404 - protein, 13 aa, Artificial Sequence
  Heavy chain CDR2 of anti-CD300c monoclonal antibody or antigen binding fragment thereof
  MISC_FEATURE (1): Xaa = T or A
  MISC_FEATURE (4): Xaa = G or S
  MISC_FEATURE (7): Xaa = T or G
  MISC_FEATURE (8): Xaa = S or Y
  MISC_FEATURE (13): Xaa = D or E
XISXSGXXTYYAX

SEQ ID NO: 405 - protein, 13 aa, Artificial Sequence
  Heavy chain CDR3 of anti-CD300c monoclonal antibody or antigen binding fragment thereof
  MISC_FEATURE (4): Xaa = R or S
  MISC_FEATURE (5): Xaa = G or S
  MISC_FEATURE (6): Xaa = M, S, Y, or I
  MISC_FEATURE (7): Xaa = W, Q, G, or R
  MISC_FEATURE (8): Xaa = G or L
  MISC_FEATURE (9): Xaa = M, I, or P
  MISC_FEATURE (10): Xaa = D, F, or L
  MISC_FEATURE (11): Xaa = V or D
  MISC_FEATURE (12): Xaa = I, Y, or not present
YCAXXXXXXXXXW

SEQ ID NO: 406 - protein, 15 aa, Artificial Sequence
  Light chain CDR1 of anti-CD300c monoclonal antibody or antigen binding fragment thereof
  MISC_FEATURE (2): Xaa = T or S
  MISC_FEATURE (3): Xaa =G or R
  MISC_FEATURE (4): Xaa = K, N, or S
  MISC_FEATURE (5): Xaa = H, N, or S
  MISC_FEATURE (6): Xaa = R, I, or G
  MISC_FEATURE (7): Xaa = H, G, or I
  MISC_FEATURE (8): Xaa = T, I, or S
  MISC_FEATURE (9): Xaa = R, A, K, or not present
  MISC_FEATURE (10): Xaa = R, S, G, or not present
  MISC_FEATURE (11): Xaa = N or not present
  MISC_FEATURE (12): Xaa = Y or not present
  MISC_FEATURE (14): Xaa = N, H, or Q
CXXXXXXXXXXXVXW

SEQ ID NO: 407 - protein, 10 aa, Artificial Sequence
  Light chain CDR2 of anti-CD300c monoclonal antibody or antigen binding fragment thereof
  MISC_FEATURE (1): Xaa = L, S, R, or E
  MISC_FEATURE (2): Xaa = D, K, or N
  MISC_FEATURE (3): Xaa = S or N
  MISC_FEATURE (4): Xaa = E, N, Q, or K
  MISC_FEATURE (10): Xaa = P or R
XXXXRPSGVX

SEQ ID NO: 408 - protein, 14 aa, Artificial Sequence
  Light chain CDR3 of anti-CD300c monoclonal antibody or antigen binding fragment thereof
  MISC_FEATURE (3): Xaa = Q, A, or S
  MISC_FEATURE (4): Xaa = S or A
  MISC_FEATURE (5): Xaa = Y or W
  MISC_FEATURE (6): Xaa = D or A
  MISC_FEATURE (7): Xaa = S, D, or G
  MISC_FEATURE (8): Xaa = S, N, or T
  MISC_FEATURE (9): Xaa = S, L, N, or K
  MISC_FEATURE (10): Xaa = V, S, N, or G
  MISC_FEATURE (11): Xaa = G, L, V, or not present
  MISC_FEATURE (12): Xaa = P or not present
YCXXXXXXXXXXVF